European Patent Specification EP 3 956 449 B1, published February 25, 2026. Title: Methods and Compositions for Editing RNAs. Applicant: EdiGene Inc. Peking University. The sequence listing filed with the application follows.

SEQUENCE LISTING (416 sequences)

SEQ ID NO: 1 - DNA, 708 bp, Artificial Sequence
  dRNA/arRNA
atggtgagcaagggcgaggaggataacatggccatcatcaaggagttcatgcgcttcaaggtgcacatggagggctccgtgaacggccacgagttcgagatcgagggcgagggcgagggccgcccctacgagggcacccagaccgccaagctgaaggtgaccaagggtggccccctgcccttcgcctgggacatcctgtcccctcagttcatgtacggctccaaggcctacgtgaagcaccccgccgacatccccgactacttgaagctgtccttccccgagggcttcaagtgggagcgcgtgatgaacttcgaggacggcggcgtggtgaccgtgacccaggactcctccctgcaggacggcgagttcatctacaaggtgaagctgcgcggcaccaacttcccctccgacggccccgtaatgcagaagaagaccatgggctgggaggcctcctccgagcggatgtaccccgaggacggcgccctgaagggcgagatcaagcagaggctgaagctgaaggacggcggccactacgacgctgaggtcaagaccacctacaaggccaagaagcccgtgcagctgcccggcgcctacaacgtcaacatcaagttggacatcacctcccacaacgaggactacaccatcgtggaacagtacgaacgcgccgagggccgccactccaccggcggcatggacgagctgtacaag

SEQ ID NO: 2 - DNA, 99 bp, Artificial Sequence
  dRNA/arRNA
ctgcagggcggaggaggcagcggcggaggaggcagcggcggaggaggcagcagaaggtatacacgccggaagaatctgtagagatccccggtcgccacc

SEQ ID NO: 3 - DNA, 717 bp, Artificial Sequence
  dRNA/arRNA
gtgagcaagggcgaggagctgttcaccggggtggtgcccatcctggtcgagctggacggcgacgtaaacggccacaagttcagcgtgtccggcgagggcgagggcgatgccacctacggcaagctgaccctgaagttcatctgcaccaccggcaagctgcccgtgccctggcccaccctcgtgaccaccctgacctacggcgtgcagtgcttcagccgctaccccgaccacatgaagcagcacgacttcttcaagtccgccatgcccgaaggctacgtccaggagcgcaccatcttcttcaaggacgacggcaactacaagacccgcgccgaggtgaagttcgagggcgacaccctggtgaaccgcatcgagctgaagggcatcgacttcaaggaggacggcaacatcctggggcacaagctggagtacaactacaacagccacaacgtctatatcatggccgacaagcagaagaacggcatcaaggtgaacttcaagatccgccacaacatcgaggacggcagcgtgcagctcgccgaccactaccagcagaacacccccatcggcgacggccccgtgctgctgcccgacaaccactacctgagcacccagtccgccctgagcaaagaccccaacgagaagcgcgatcacatggtcctgctggagttcgtgaccgccgccgggatcactctcggcatggacgagctgtacaagtaa

SEQ ID NO: 4 - DNA, 81 bp, Artificial Sequence
  dRNA/arRNA
ctgcagggcggaggaggcagcggcggaggaggcagcggcggaggaggcagcgcctgctcgcgatgctagagggctctgcca

SEQ ID NO: 5 - DNA, 50 bp, Artificial Sequence
  dRNA/arRNA
ctgcagggcggaggaggcagcgcctgctcgcgatgctagagggctctgcc

SEQ ID NO: 6 - RNA, 101 nt, Artificial Sequence
  dRNA/arRNA
ggaccaccccaaaaaugaauauaaccaaaacugaacagcuccucgcccuugcucacuggcagagcccuccagcaucgcgagcaggcgcugccuccuccgcc

SEQ ID NO: 7 - RNA, 70 nt, Artificial Sequence
  dRNA/arRNA
aaaccgagggaucauaggggacugaauccaccauucuucucccaaucccugcaacuccuucuuccccugc

SEQ ID NO: 8 - RNA, 70 nt, Artificial Sequence
  dRNA/arRNA
ugaacagcuccucgcccuugcucacuggcagagcccuccagcaucgcgagcaggcgcugccuccuccgcc

SEQ ID NO: 9 - DNA, 111 bp, Artificial Sequence
  dRNA/arRNA
atggacgagctgtacaagctgcagggcggaggaggcagcgcctgctcgcgatgctatagggctctgccagtgagcaagggcgaggagctgttcaccggggtggtgcccatc

SEQ ID NO: 10 - DNA, 111 bp, Artificial Sequence
  dRNA/arRNA
atggacgagctgtacaagctgcagggcggaggaggcagcgcctgctcgcgatgctaaagggctctgccagtgagcaagggcgaggagctgttcaccggggtggtgcccatc

SEQ ID NO: 11 - DNA, 111 bp, Artificial Sequence
  dRNA/arRNA
atggacgagctgtacaagctgcagggcggaggaggcagcgcctgctcgcgatgctacagggctctgccagtgagcaagggcgaggagctgttcaccggggtggtgcccatc

SEQ ID NO: 12 - DNA, 111 bp, Artificial Sequence
  dRNA/arRNA
atggacgagctgtacaagctgcagggcggaggaggcagcgcctgctcgcgatgctagagggctctgccagtgagcaagggcgaggagctgttcaccggggtggtgcccatc

SEQ ID NO: 13 - DNA, 111 bp, Artificial Sequence
  dRNA/arRNA
atggacgagctgtacaagctgcagggcggaggaggcagcgcctgctcgcgatgcaatagggctctgccagtgagcaagggcgaggagctgttcaccggggtggtgcccatc

SEQ ID NO: 14 - DNA, 111 bp, Artificial Sequence
  dRNA/arRNA
atggacgagctgtacaagctgcagggcggaggaggcagcgcctgctcgcgatgcaaaagggctctgccagtgagcaagggcgaggagctgttcaccggggtggtgcccatc

SEQ ID NO: 15 - DNA, 111 bp, Artificial Sequence
  dRNA/arRNA
atggacgagctgtacaagctgcagggcggaggaggcagcgcctgctcgcgatgcaacagggctctgccagtgagcaagggcgaggagctgttcaccggggtggtgcccatc

SEQ ID NO: 16 - DNA, 111 bp, Artificial Sequence
  dRNA/arRNA
atggacgagctgtacaagctgcagggcggaggaggcagcgcctgctcgcgatgcaagagggctctgccagtgagcaagggcgaggagctgttcaccggggtggtgcccatc

SEQ ID NO: 17 - DNA, 111 bp, Artificial Sequence
  dRNA/arRNA
atggacgagctgtacaagctgcagggcggaggaggcagcgcctgctcgcgatgccatagggctctgccagtgagcaagggcgaggagctgttcaccggggtggtgcccatc

SEQ ID NO: 18 - DNA, 111 bp, Artificial Sequence
  dRNA/arRNA
atggacgagctgtacaagctgcagggcggaggaggcagcgcctgctcgcgatgccaaagggctctgccagtgagcaagggcgaggagctgttcaccggggtggtgcccatc

SEQ ID NO: 19 - DNA, 111 bp, Artificial Sequence
  dRNA/arRNA
atggacgagctgtacaagctgcagggcggaggaggcagcgcctgctcgcgatgccacagggctctgccagtgagcaagggcgaggagctgttcaccggggtggtgcccatc

SEQ ID NO: 20 - DNA, 111 bp, Artificial Sequence
  dRNA/arRNA
atggacgagctgtacaagctgcagggcggaggaggcagcgcctgctcgcgatgccagagggctctgccagtgagcaagggcgaggagctgttcaccggggtggtgcccatc

SEQ ID NO: 21 - DNA, 111 bp, Artificial Sequence
  dRNA/arRNA
atggacgagctgtacaagctgcagggcggaggaggcagcgcctgctcgcgatgcgatagggctctgccagtgagcaagggcgaggagctgttcaccggggtggtgcccatc

SEQ ID NO: 22 - DNA, 111 bp, Artificial Sequence
  dRNA/arRNA
atggacgagctgtacaagctgcagggcggaggaggcagcgcctgctcgcgatgcgaaagggctctgccagtgagcaagggcgaggagctgttcaccggggtggtgcccatc

SEQ ID NO: 23 - DNA, 111 bp, Artificial Sequence
  dRNA/arRNA
atggacgagctgtacaagctgcagggcggaggaggcagcgcctgctcgcgatgcgacagggctctgccagtgagcaagggcgaggagctgttcaccggggtggtgcccatc

SEQ ID NO: 24 - DNA, 111 bp, Artificial Sequence
  dRNA/arRNA
atggacgagctgtacaagctgcagggcggaggaggcagcgcctgctcgcgatgcgagagggctctgccagtgagcaagggcgaggagctgttcaccggggtggtgcccatc

SEQ ID NO: 25 - RNA, 91 nt, Artificial Sequence
  dRNA/arRNA
uagcuguaucgucaaggcacucuugccuacgccaccagcuccaaccaccacaaguuuauauucagucauuuucagcaggccucucucccgc

SEQ ID NO: 26 - RNA, 111 nt, Artificial Sequence
  dRNA/arRNA
gauucugaauuagcuguaucgucaaggcacucuugccuacgccaccagcuccaacuaccacaaguuuauauucagucauuuucagcaggccucucucccgcaccugggagc

SEQ ID NO: 27 - RNA, 131 nt, Artificial Sequence
  dRNA/arRNA
uccacaaaaugauucugaauuagcuguaucgucaaggcacucuugccuacgccaccagcuccaacuaccacaaguuuauauucagucauuuucagcaggccucucucccgcaccugggagccgcugagccu

SEQ ID NO: 28 - RNA, 151 nt, Artificial Sequence
  dRNA/arRNA
aucauauucguccacaaaaugauucugaauuagcuguaucgucaaggcacucuugccuacgccaccagcuccaaccaccacaaguuuauauucagucauuuucagcaggccucucucccgcaccugggagccgcugagccucuggccccgc

SEQ ID NO: 29 - RNA, 171 nt, Artificial Sequence
  dRNA/arRNA
cuauuguuggaucauauucguccacaaaaugauucugaauuagcuguaucgucaaggcacucuugccuacgccaccagcuccaaccaccacaaguuuauauucagucauuuucagcaggccucucucccgcaccugggagccgcugagccucuggccccgccgccgccuuc

SEQ ID NO: 30 - RNA, 191 nt, Artificial Sequence
  dRNA/arRNA
uaggaauccucuauuguuggaucauauucguccacaaaaugauucugaauuagcuguaucgucaaggcacucuugccuacgccaccagcuccaaccaccacaaguuuauauucagucauuuucagcaggccucucucccgcaccugggagccgcugagccucuggccccgccgccgccuucagugccugcg

SEQ ID NO: 31 - RNA, 151 nt, Artificial Sequence
  dRNA/arRNA
gaggcgcagcauccacaggcggaggcgaaagcagcccggacagcugaggccggaagaggguggggccgcgguggccagggagccggcgccgccacgcgcgggugggggggacugggguugcucgcgggcuccgggcgggcggcgggcgccg

SEQ ID NO: 32 - RNA, 151 nt, Artificial Sequence
  dRNA/arRNA
uccuguagcuaaggccacaaaauuauccacuguuuuuggaacagucuuuccgaagagaccaaagaucacccggcccacaucuucaucuccaauucguaggucaaaauacaccuugacggugacuuugggccccuucuucuucucaucggcc

SEQ ID NO: 33 - RNA, 151 nt, Artificial Sequence
  dRNA/arRNA
gcccuggaucaugaaguccuugauuacacgauggaauuugcuguuuuuguagccaaauccuuucucuccuguagccaaggccacaaaauuauccacuguuuuuggaacagucuuuccgaagagaccaaagaucacccggccuacaucuuca

SEQ ID NO: 34 - RNA, 72 nt, Artificial Sequence
  dRNA/arRNA
gcgcaaguuagguuuugucaagaaaggguguaacgcaaccaagucauaguccgccuagaagcauuugcggug

SEQ ID NO: 35 - RNA, 131 nt, Artificial Sequence
  dRNA/arRNA
gccaugccaaucucaucuuguuuucugcgcaaguuagguuuugucaagaaaggguguaacgcaaccaagucauaguccgccuagaagcauuugcgguggacgauggaggggccggacucgucauacuccug

SEQ ID NO: 36 - RNA, 70 nt, Artificial Sequence
  dRNA/arRNA
ggacuuccuguaacaacgcaucucauauuuggaaugaccauuaaaaaaacaacaaugugcaaucaaaguc

SEQ ID NO: 37 - RNA, 71 nt, Artificial Sequence
  dRNA/arRNA
caaggugcggcuccggccccuccccucuucaagggguccacauggcaacugugaggaggggagauucagug

SEQ ID NO: 38 - RNA, 91 nt, Artificial Sequence
  dRNA/arRNA
uagcuguaucgucaaggcacucgugccgacgccaccagcuccaaccaccacaaggggagagucagucagggucagcaggccucucucccgc

SEQ ID NO: 39 - RNA, 91 nt, Artificial Sequence
  dRNA/arRNA
uagcuguaucgucaaggcacucuugccgacgccaccagcuccaaccaccacaaguguauagucagucauuuucagcaggccucucucccgc

SEQ ID NO: 40 - RNA, 91 nt, Artificial Sequence
  dRNA/arRNA
uagcuggaucgucaaggcacucgugccgacgccaccagcuccaaccaccacaaggggagaggcagucagggucagcaggccucucucccgc

SEQ ID NO: 41 - RNA, 111 nt, Artificial Sequence
  dRNA/arRNA
gauucugaauuagcuguaucgucaaggcacucuugccgacgccaccagcuccaaccaccacaaguguauagucagucauuuucagcaggccucucucccgcaccugggagc

SEQ ID NO: 42 - RNA, 111 nt, Artificial Sequence
  dRNA/arRNA
gauucugaauuagcuguaucgucaaggcacucgugccgacgccaccagcuccaaccaccacaaguggagagucagucauuuucagcaggccucucucccgcaccugggagc

SEQ ID NO: 43 - RNA, 111 nt, Artificial Sequence
  dRNA/arRNA
gauucugaauuagcuguaucgucaaggcacucgugccgacgccaccagcuccaaccaccacaaggggagagucagucagggucagcaggccucucucccgcaccugggagc

SEQ ID NO: 44 - RNA, 111 nt, Artificial Sequence
  dRNA/arRNA
gcuccccggugcgggagagaggccugcugacccugacugccucuccccuuguggugguuggagcugguggcgucggcacgagugccuugacgauccagcuaauucagaauc

SEQ ID NO: 45 - DNA, 71 bp, Artificial Sequence
  dRNA/arRNA
tctcagtccaatgtatggtccgagcacaagctctaatcaaagtccgcgggtgtagaccggttgccatagga

SEQ ID NO: 46 - RNA, 31 nt, Artificial Sequence
  dRNA/arRNA
ggaccaccccaaaaaugaaggggacuaaaac

SEQ ID NO: 47 - RNA, 70 nt, Artificial Sequence; identical to SEQ ID NO: 7
  dRNA/arRNA

SEQ ID NO: 48 - RNA, 14 nt, Artificial Sequence
  dRNA/arRNA
gcagagccuccagc

SEQ ID NO: 49 - RNA, 21 nt, Artificial Sequence
  dRNA/arRNA
cucacuggcagagccuccagc

SEQ ID NO: 50 - RNA, 27 nt, Artificial Sequence
  dRNA/arRNA
cccuugcucacuggcagagccuccagc

SEQ ID NO: 51 - RNA, 33 nt, Artificial Sequence
  dRNA/arRNA
cucucgcccuugcucacuggcagagccuccagc

SEQ ID NO: 52 - RNA, 38 nt, Artificial Sequence
  dRNA/arRNA
cucucgcccuugcucacuggcagagccuccagcaucgc

SEQ ID NO: 53 - RNA, 45 nt, Artificial Sequence
  dRNA/arRNA
ugaacagcucucgcccuugcucacuggcagagccuccagcaucgc

SEQ ID NO: 54 - RNA, 70 nt, Artificial Sequence; identical to SEQ ID NO: 8
  dRNA/arRNA

SEQ ID NO: 55 - RNA, 70 nt, Artificial Sequence; identical to SEQ ID NO: 7
  dRNA/arRNA

SEQ ID NO: 56 - RNA, 70 nt, Artificial Sequence; identical to SEQ ID NO: 8
  dRNA/arRNA

SEQ ID NO: 57 - RNA, 71 nt, Artificial Sequence
  dRNA/arRNA
ucucaguccaauguaugguccgagcacaagcucuaaucaaaguccgcggguguagaccgguugccauagga

SEQ ID NO: 58 - RNA, 71 nt, Artificial Sequence
  dRNA/arRNA
acagcuccucgcccuugcucacuggcagagcccuccagcaucgcgagcaggcgcugccuccuccgccgcug

SEQ ID NO: 59 - RNA, 71 nt, Artificial Sequence
  dRNA/arRNA
acagcuccucgcccuugcucacuggcagagcccucaagcaucgcgagcaggcgcugccuccuccgccgcug

SEQ ID NO: 60 - RNA, 71 nt, Artificial Sequence
  dRNA/arRNA
acagcuccucgcccuugcucacuggcagagcccucuagcaucgcgagcaggcgcugccuccuccgccgcug

SEQ ID NO: 61 - RNA, 71 nt, Artificial Sequence
  dRNA/arRNA
acagcuccucgcccuugcucacuggcagagcccucgagcaucgcgagcaggcgcugccuccuccgccgcug

SEQ ID NO: 62 - RNA, 71 nt, Artificial Sequence
  dRNA/arRNA
acagcuccucgcccuugcucacuggcagagcccugcagcaucgcgagcaggcgcugccuccuccgccgcug

SEQ ID NO: 63 - RNA, 71 nt, Artificial Sequence
  dRNA/arRNA
acagcuccucgcccuugcucacuggcagagcccuucagcaucgcgagcaggcgcugccuccuccgccgcug

SEQ ID NO: 64 - RNA, 71 nt, Artificial Sequence
  dRNA/arRNA
acagcuccucgcccuugcucacuggcagagcccuacagcaucgcgagcaggcgcugccuccuccgccgcug

SEQ ID NO: 65 - RNA, 71 nt, Artificial Sequence
  dRNA/arRNA
acagcuccucgcccuugcucacuggcagagcccuccugcaucgcgagcaggcgcugccuccuccgccgcug

SEQ ID NO: 66 - RNA, 71 nt, Artificial Sequence
  dRNA/arRNA
acagcuccucgcccuugcucacuggcagagcccugcugcaucgcgagcaggcgcugccuccuccgccgcug

SEQ ID NO: 67 - RNA, 71 nt, Artificial Sequence
  dRNA/arRNA
acagcuccucgcccuugcucacuggcagagcccuucugcaucgcgagcaggcgcugccuccuccgccgcug

SEQ ID NO: 68 - RNA, 71 nt, Artificial Sequence
  dRNA/arRNA
acagcuccucgcccuugcucacuggcagagcccuacugcaucgcgagcaggcgcugccuccuccgccgcug

SEQ ID NO: 69 - RNA, 71 nt, Artificial Sequence
  dRNA/arRNA
acagcuccucgcccuugcucacuggcagagcccucccgcaucgcgagcaggcgcugccuccuccgccgcug

SEQ ID NO: 70 - RNA, 71 nt, Artificial Sequence
  dRNA/arRNA
acagcuccucgcccuugcucacuggcagagcccugccgcaucgcgagcaggcgcugccuccuccgccgcug

SEQ ID NO: 71 - RNA, 71 nt, Artificial Sequence
  dRNA/arRNA
acagcuccucgcccuugcucacuggcagagcccuuccgcaucgcgagcaggcgcugccuccuccgccgcug

SEQ ID NO: 72 - RNA, 71 nt, Artificial Sequence
  dRNA/arRNA
acagcuccucgcccuugcucacuggcagagcccuaccgcaucgcgagcaggcgcugccuccuccgccgcug

SEQ ID NO: 73 - RNA, 71 nt, Artificial Sequence
  dRNA/arRNA
acagcuccucgcccuugcucacuggcagagcccuccggcaucgcgagcaggcgcugccuccuccgccgcug

SEQ ID NO: 74 - RNA, 71 nt, Artificial Sequence; identical to SEQ ID NO: 66
  dRNA/arRNA

SEQ ID NO: 75 - RNA, 71 nt, Artificial Sequence
  dRNA/arRNA
acagcuccucgcccuugcucacuggcagagcccuucggcaucgcgagcaggcgcugccuccuccgccgcug

SEQ ID NO: 76 - RNA, 71 nt, Artificial Sequence
  dRNA/arRNA
acagcuccucgcccuugcucacuggcagagcccuacggcaucgcgagcaggcgcugccuccuccgccgcug

SEQ ID NO: 77 - RNA, 31 nt, Artificial Sequence
  dRNA/arRNA
acuggcagagcccuccagcaucgcgagcagg

SEQ ID NO: 78 - RNA, 51 nt, Artificial Sequence
  dRNA/arRNA
gcccuugcucacuggcagagcccuccagcaucgcgagcaggcgcugccucc

SEQ ID NO: 79 - RNA, 71 nt, Artificial Sequence; identical to SEQ ID NO: 58
  dRNA/arRNA

SEQ ID NO: 80 - RNA, 91 nt, Artificial Sequence
  dRNA/arRNA
accccggugaacagcuccucgcccuugcucacuggcagagcccuccagcaucgcgagcaggcgcugccuccuccgccgcugccuccuccgc

SEQ ID NO: 81 - RNA, 131 nt, Artificial Sequence
  dRNA/arRNA
gcucgaccaggaugggcaccaccccggugaacagcuccucgcccuugcucacuggcagagcccuccagcaucgcgagcaggcgcugccuccuccgccgcugccuccuccgccgcugccuccuccgcccugc

SEQ ID NO: 82 - RNA, 151 nt, Artificial Sequence
  dRNA/arRNA
ucgccguccagcucgaccaggaugggcaccaccccggugaacagcuccucgcccuugcucacuggcagagcccuccagcaucgcgagcaggcgcugccuccuccgccgcugccuccuccgccgcugccuccuccgcccugcagcuuguaca

SEQ ID NO: 83 - RNA, 171 nt, Artificial Sequence
  dRNA/arRNA
gccguuuacgucgccguccagcucgaccaggaugggcaccaccccggugaacagcuccucgcccuugcucacuggcagagcccuccagcaucgcgagcaggcgcugccuccuccgccgcugccuccuccgccgcugccuccuccgcccugcagcuuguacagcucguccau

SEQ ID NO: 84 - RNA, 191 nt, Artificial Sequence
  dRNA/arRNA
ugaacuuguggccguuuacgucgccguccagcucgaccaggaugggcaccaccccggugaacagcuccucgcccuugcucacuggcagagcccuccagcaucgcgagcaggcgcugccuccuccgccgcugccuccuccgccgcugccuccuccgcccugcagcuuguacagcucguccaugccgccggug

SEQ ID NO: 85 - RNA, 211 nt, Artificial Sequence
  dRNA/arRNA
ccggacacgcugaacuuguggccguuuacgucgccguccagcucgaccaggaugggcaccaccccggugaacagcuccucgcccuugcucacuggcagagcccuccagcaucgcgagcaggcgcugccuccuccgccgcugccuccuccgccgcugccuccuccgcccugcagcuuguacagcucguccaugccgccgguggaguggcggc

SEQ ID NO: 86 - RNA, 31 nt, Artificial Sequence
  dRNA/arRNA
gcgaccggggaucuccacagauucuuccggc

SEQ ID NO: 87 - RNA, 51 nt, Artificial Sequence
  dRNA/arRNA
gcucacgguggcgaccggggaucuccacagauucuuccggcguguauaccu

SEQ ID NO: 88 - RNA, 71 nt, Artificial Sequence
  dRNA/arRNA
ccucgcccuugcucacgguggcgaccggggaucuccacagauucuuccggcguguauaccuucugcugccu

SEQ ID NO: 89 - RNA, 91 nt, Artificial Sequence
  dRNA/arRNA
gugaacagcuccucgcccuugcucacgguggcgaccggggaucuccacagauucuuccggcguguauaccuucugcugccuccuccgccgc

SEQ ID NO: 90 - RNA, 111 nt, Artificial Sequence
  dRNA/arRNA
caccaccccggugaacagcuccucgcccuugcucacgguggcgaccggggaucuccacagauucuuccggcguguauaccuucugcugccuccuccgccgcugccuccucc

SEQ ID NO: 91 - RNA, 131 nt, Artificial Sequence
  dRNA/arRNA
ccaggaugggcaccaccccggugaacagcuccucgcccuugcucacgguggcgaccggggaucuccacagauucuuccggcguguauaccuucugcugccuccuccgccgcugccuccuccgccgcugccu

SEQ ID NO: 92 - RNA, 151 nt, Artificial Sequence
  dRNA/arRNA
uccagcucgaccaggaugggcaccaccccggugaacagcuccucgcccuugcucacgguggcgaccggggaucuccacagauucuuccggcguguauaccuucugcugccuccuccgccgcugccuccuccgccgcugccuccuccgcccu

SEQ ID NO: 93 - RNA, 171 nt, Artificial Sequence
  dRNA/arRNA
cggcgacguauccagcucgaccaggaugggcaccaccccggugaacagcuccucgcccuugcucacgguggcgaccggggaucuccacagauucuuccggcguguauaccuucugcugccuccuccgccgcugccuccuccgccgcugccuccuccgcccugcagcuugua

SEQ ID NO: 94 - RNA, 191 nt, Artificial Sequence
  dRNA/arRNA
uguggccguuuacgucgccguccagcucgaccaggaugggcaccaccccggugaacagcuccucgcccuugcucacgguggcgaccggggaucuccacagauucuuccggcguguauaccuucugcugccuccuccgccgcugccuccuccgccgcugccuccuccgcccugcagcuuguacagcucgucc

SEQ ID NO: 95 - RNA, 211 nt, Artificial Sequence
  dRNA/arRNA
acgcugaacuuguggccguuuacgucgccguccagcucgaccaggaugggcaccaccccggugaacagcuccucgcccuugcucacgguggcgaccggggaucuccacagauucuuccggcguguauaccuucugcugccuccuccgccgcugccuccuccgccgcugccuccuccgcccugcagcuuguacagcucguccaugccgccgg

SEQ ID NO: 96 - RNA, 71 nt, Artificial Sequence
  dRNA/arRNA
cagcaucgcgagcaggcgcugccuccuccgccgcugccuccuccgccgcugccuccuccgcccugcagcuu

SEQ ID NO: 97 - RNA, 71 nt, Artificial Sequence
  dRNA/arRNA
cccuccagcaucgcgagcaggcgcugccuccuccgccgcugccuccuccgccgcugccuccuccgcccugc

SEQ ID NO: 98 - RNA, 71 nt, Artificial Sequence
  dRNA/arRNA
cagagcccuccagcaucgcgagcaggcgcugccuccuccgccgcugccuccuccgccgcugccuccuccgc

SEQ ID NO: 99 - RNA, 72 nt, Artificial Sequence
  dRNA/arRNA
acuggcagagcccucccagcaucgcgagcaggcgcugccuccuccgccgcugccuccuccgccgcugccucc

SEQ ID NO: 100 - RNA, 71 nt, Artificial Sequence
  dRNA/arRNA
ugcucacuggcagagcccuccagcaucgcgagcaggcgcugccuccuccgccgcugccuccuccgccgcug

SEQ ID NO: 101 - RNA, 71 nt, Artificial Sequence
  dRNA/arRNA
gcccuugcucacuggcagagcccuccagcaucgcgagcaggcgcugccuccuccgccgcugccuccuccgc

SEQ ID NO: 102 - RNA, 71 nt, Artificial Sequence
  dRNA/arRNA
uccucgcccuugcucacuggcagagcccuccagcaucgcgagcaggcgcugccuccuccgccgcugccucc

SEQ ID NO: 103 - RNA, 71 nt, Artificial Sequence
  dRNA/arRNA
ggugaacagcuccucgcccuugcucacuggcagagcccuccagcaucgcgagcaggcgcugccuccuccgc

SEQ ID NO: 104 - RNA, 71 nt, Artificial Sequence
  dRNA/arRNA
accccggugaacagcuccucgcccuugcucacuggcagagcccuccagcaucgcgagcaggcgcugccucc

SEQ ID NO: 105 - RNA, 71 nt, Artificial Sequence
  dRNA/arRNA
gcaccaccccggugaacagcuccucgcccuugcucacuggcagagcccuccagcaucgcgagcaggcgcug

SEQ ID NO: 106 - RNA, 71 nt, Artificial Sequence
  dRNA/arRNA
gaugggcaccaccccggugaacagcuccucgcccuugcucacuggcagagcccuccagcaucgcgagcagg

SEQ ID NO: 107 - RNA, 71 nt, Artificial Sequence
  dRNA/arRNA
accaggaugggcaccaccccggugaacagcuccucgcccuugcucacuggcagagcccuccagcaucgcga

SEQ ID NO: 108 - RNA, 71 nt, Artificial Sequence
  dRNA/arRNA
gcucgaccaggaugggcaccaccccggugaacagcuccucgcccuugcucacuggcagagcccuccagcau

SEQ ID NO: 109 - RNA, 71 nt, Artificial Sequence
  dRNA/arRNA
guccagcucgaccaggaugggcaccaccccggugaacagcuccucgcccuugcucacuggcagagcccucc

SEQ ID NO: 110 - RNA, 71 nt, Artificial Sequence
  dRNA/arRNA
cacagauucuuccggcguguauaccuucugcugccuccuccgccgcugccuccuccgccgcugccuccucc

SEQ ID NO: 111 - RNA, 71 nt, Artificial Sequence
  dRNA/arRNA
aucuccacagauucuuccggcguguauaccuucugcugccuccuccgccgcugccuccuccgccgcugccu

SEQ ID NO: 112 - RNA, 71 nt, Artificial Sequence
  dRNA/arRNA
cggggaucuccacagauucuuccggcguguauaccuucugcugccuccuccgccgcugccuccuccgccgc

SEQ ID NO: 113 - RNA, 71 nt, Artificial Sequence
  dRNA/arRNA
gcgaccggggaucuccacagauucuuccggcguguauaccuucugcugccuccuccgccgcugccuccucc

SEQ ID NO: 114 - RNA, 71 nt, Artificial Sequence
  dRNA/arRNA
cgguggcgaccggggaucuccacagauucuuccggcguguauaccuucugcugccuccuccgccgcugccu

SEQ ID NO: 115 - RNA, 71 nt, Artificial Sequence
  dRNA/arRNA
gcucacgguggcgaccggggaucuccacagauucuuccggcguguauaccuucugcugccuccuccgccgc

SEQ ID NO: 116 - RNA, 71 nt, Artificial Sequence
  dRNA/arRNA
cccuugcucacgguggcgaccggggaucuccacagauucuuccggcguguauaccuucugcugccuccucc

SEQ ID NO: 117 - RNA, 71 nt, Artificial Sequence
  dRNA/arRNA
cagcuccucgcccuugcucacgguggcgaccggggaucuccacagauucuuccggcguguauaccuucugc

SEQ ID NO: 118 - RNA, 71 nt, Artificial Sequence
  dRNA/arRNA
gugaacagcuccucgcccuugcucacgguggcgaccggggaucuccacagauucuuccggcguguauaccu

SEQ ID NO: 119 - RNA, 71 nt, Artificial Sequence
  dRNA/arRNA
ccccggugaacagcuccucgcccuugcucacgguggcgaccggggaucuccacagauucuuccggcgugua

SEQ ID NO: 120 - RNA, 71 nt, Artificial Sequence
  dRNA/arRNA
caccaccccggugaacagcuccucgcccuugcucacgguggcgaccggggaucuccacagauucuuccggc

SEQ ID NO: 121 - RNA, 71 nt, Artificial Sequence
  dRNA/arRNA
augggcaccaccccggugaacagcuccucgcccuugcucacgguggcgaccggggaucuccacagauucuu

SEQ ID NO: 122 - RNA, 71 nt, Artificial Sequence
  dRNA/arRNA
ccaggaugggcaccaccccggugaacagcuccucgcccuugcucacgguggcgaccggggaucuccacaga

SEQ ID NO: 123 - RNA, 71 nt, Artificial Sequence
  dRNA/arRNA
cucgaccaggaugggcaccaccccggugaacagcuccucgcccuugcucacgguggcgaccggggaucucc

SEQ ID NO: 124 - RNA, 111 nt, Artificial Sequence
  dRNA/arRNA
gaugggcaccaccccggugaacagcuccucgcccuugcucacuggcagagcccuccagcaucgcgagcaggcgcugccuccuccgcccugcagcuuguacagcucguccau

SEQ ID NO: 125 - RNA, 111 nt, Artificial Sequence
  dRNA/arRNA
gaugggcaccaccccggugaacagcuccucgcccuugcucacuggcagagcccugcagcaucgcgagcaggcgcugccuccuccgcccugcagcuuguacagcucguccau

SEQ ID NO: 126 - RNA, 111 nt, Artificial Sequence
  dRNA/arRNA
gaugggcaccaccccggugaacagcuccucgcccuugcucacuggcagagcccuucagcaucgcgagcaggcgcugccuccuccgcccugcagcuuguacagcucguccau

SEQ ID NO: 127 - RNA, 111 nt, Artificial Sequence
  dRNA/arRNA
gaugggcaccaccccggugaacagcuccucgcccuugcucacuggcagagcccuacagcaucgcgagcaggcgcugccuccuccgcccugcagcuuguacagcucguccau

SEQ ID NO: 128 - RNA, 111 nt, Artificial Sequence
  dRNA/arRNA
gaugggcaccaccccggugaacagcuccucgcccuugcucacuggcagagcccuccggcaucgcgagcaggcgcugccuccuccgcccugcagcuuguacagcucguccau

SEQ ID NO: 129 - RNA, 111 nt, Artificial Sequence
  dRNA/arRNA
gaugggcaccaccccggugaacagcuccucgcccuugcucacuggcagagcccugcggcaucgcgagcaggcgcugccuccuccgcccugcagcuuguacagcucguccau

SEQ ID NO: 130 - RNA, 111 nt, Artificial Sequence
  dRNA/arRNA
gaugggcaccaccccggugaacagcuccucgcccuugcucacuggcagagcccuucggcaucgcgagcaggcgcugccuccuccgcccugcagcuuguacagcucguccau

SEQ ID NO: 131 - RNA, 111 nt, Artificial Sequence
  dRNA/arRNA
gaugggcaccaccccggugaacagcuccucgcccuugcucacuggcagagcccuacggcaucgcgagcaggcgcugccuccuccgcccugcagcuuguacagcucguccau

SEQ ID NO: 132 - RNA, 111 nt, Artificial Sequence
  dRNA/arRNA
gaugggcaccaccccggugaacagcuccucgcccuugcucacuggcagagcccuccugcaucgcgagcaggcgcugccuccuccgcccugcagcuuguacagcucguccau

SEQ ID NO: 133 - RNA, 111 nt, Artificial Sequence
  dRNA/arRNA
gaugggcaccaccccggugaacagcuccucgcccuugcucacuggcagagcccugcugcaucgcgagcaggcgcugccuccuccgcccugcagcuuguacagcucguccau

SEQ ID NO: 134 - RNA, 111 nt, Artificial Sequence
  dRNA/arRNA
gaugggcaccaccccggugaacagcuccucgcccuugcucacuggcagagcccuacugcaucgcgagcaggcgcugccuccuccgcccugcagcuuguacagcucguccau

SEQ ID NO: 135 - RNA, 111 nt, Artificial Sequence
  dRNA/arRNA
gaugggcaccaccccggugaacagcuccucgcccuugcucacuggcagagcccuucugcaucgcgagcaggcgcugccuccuccgcccugcagcuuguacagcucguccau

SEQ ID NO: 136 - RNA, 111 nt, Artificial Sequence
  dRNA/arRNA
gaugggcaccaccccggugaacagcuccucgcccuugcucacuggcagagcccucccgcaucgcgagcaggcgcugccuccuccgcccugcagcuuguacagcucguccau

SEQ ID NO: 137 - RNA, 111 nt, Artificial Sequence
  dRNA/arRNA
gaugggcaccaccccggugaacagcuccucgcccuugcucacuggcagagcccugccgcaucgcgagcaggcgcugccuccuccgcccugcagcuuguacagcucguccau

SEQ ID NO: 138 - RNA, 111 nt, Artificial Sequence
  dRNA/arRNA
gaugggcaccaccccggugaacagcuccucgcccuugcucacuggcagagcccuuccgcaucgcgagcaggcgcugccuccuccgcccugcagcuuguacagcucguccau

SEQ ID NO: 139 - RNA, 111 nt, Artificial Sequence
  dRNA/arRNA
gaugggcaccaccccggugaacagcuccucgcccuugcucacuggcagagcccuaccgcaucgcgagcaggcgcugccuccuccgcccugcagcuuguacagcucguccau

SEQ ID NO: 140 - RNA, 111 nt, Artificial Sequence
  dRNA/arRNA
uaccgcuacagccacgcugauuucagcuauaccugcccgguauaaagggacguucacaccgcgauguucucugcuggggaauugcgcgauauucaggauuaaaagaagugc

SEQ ID NO: 141 - RNA, 151 nt, Artificial Sequence
  dRNA/arRNA
acuacaguugcuccgauauuuaggcuacgucaauaggcacuaacuuauuggcgcuggugaacggacuuccucucgaguaccagaagaugacuacaaaacuccuuuccauugcgaguaucggagucuggcucaguuuggccagggaggcacu

SEQ ID NO: 142 - RNA, 51 nt, Artificial Sequence
  dRNA/arRNA
cggaagaggguggggccgcgguggccagggagccggcgccgccacgcgcgg

SEQ ID NO: 143 - RNA, 71 nt, Artificial Sequence
  dRNA/arRNA
cagcugaggccggaagaggguggggccgcgguggccagggagccggcgccgccacgcgcggguggggggga

SEQ ID NO: 144 - RNA, 111 nt, Artificial Sequence
  dRNA/arRNA
ggaggcgaaagcagcccggacagcugaggccggaagaggguggggccgcgguggccagggagccggcgccgccacgcgcgggugggggggacugggguugcucgcgggcuc

SEQ ID NO: 145 - RNA, 151 nt, Artificial Sequence; identical to SEQ ID NO: 31
  dRNA/arRNA

SEQ ID NO: 146 - RNA, 51 nt, Artificial Sequence
  dRNA/arRNA
ucuugccuacgccaccagcuccaaccaccacaaguuuauauucagucauuu

SEQ ID NO: 147 - RNA, 111 nt, Artificial Sequence
  dRNA/arRNA
gauucugaauuagcuguaucgucaaggcacucuugccuacgccaccagcuccaaccaccacaaguuuauauucagucauuuucagcaggccucucucccgcaccugggagc

SEQ ID NO: 148 - RNA, 151 nt, Artificial Sequence; identical to SEQ ID NO: 28
  dRNA/arRNA

SEQ ID NO: 149 - RNA, 51 nt, Artificial Sequence
  dRNA/arRNA
ucggcaugguaugaaguacuucguccaggagcuggagggcccgguguaagu

SEQ ID NO: 150 - RNA, 71 nt, Artificial Sequence
  dRNA/arRNA
gggucugcaaucggcaugguaugaaguacuucguccaggagcuggagggcccgguguaagugaauuucaau

SEQ ID NO: 151 - RNA, 111 nt, Artificial Sequence
  dRNA/arRNA
gaccucagucuaaagguugugggucugcaaucggcaugguaugaaguacuucguccaggagcuggagggcccgguguaagugaauuucaauccagcaagguguuucuuuga

SEQ ID NO: 152 - RNA, 151 nt, Artificial Sequence
  dRNA/arRNA
uaagggccccaacgguaaaagaccucagucuaaagguugugggucugcaaucggcaugguaugaaguacuucguccaggagcuggagggcccgguguaagugaauuucaauccagcaagguguuucuuugaugcucugucuuggguaaucc

SEQ ID NO: 153 - RNA, 51 nt, Artificial Sequence
  dRNA/arRNA
ugggggguucggcugccgacaucagcaauugcucugccaccaucucagccc

SEQ ID NO: 154 - RNA, 71 nt, Artificial Sequence
  dRNA/arRNA
agcagggccgugggggguucggcugccgacaucagcaauugcucugccaccaucucagcccauccuccgaa

SEQ ID NO: 155 - RNA, 111 nt, Artificial Sequence
  dRNA/arRNA
aguagaaggccaagagccacagcagggccgugggggguucggcugccgacaucagcaauugcucugccaccaucucagcccauccuccgaagugaaugaacaggaaccagc

SEQ ID NO: 156 - RNA, 151 nt, Artificial Sequence
  dRNA/arRNA
ccucccaucacgggggccguaguagaaggccaagagccacagcagggccgugggggguucggcugccgacaucagcaauugcucugccaccaucucagcccauccuccgaagugaaugaacaggaaccagcucucaaagggaccuccgcag

SEQ ID NO: 157 - DNA, 151 bp, Artificial Sequence
  dRNA/arRNA
gccaaacaccacatgcttgccatctagccaggctgtcttgactgtcgtgatgaagaactgggagccgttggtgtccttgcctgcgttggccatgctcacccagccaggcccgtagtgcttcagtttgaagttctcatcggggaagcgctca

SEQ ID NO: 158 - DNA, 151 bp, Artificial Sequence
  dRNA/arRNA
gggagtgggtccgctccaccagatgccagcaccggggccagtgcagctcagagccctgtggcggactacagggcccgcacagacggtcactcaaagaaagatgtccctgtgccctactccttggcgatggcaaagggcttctccacctcga

SEQ ID NO: 159 - DNA, 151 bp, Artificial Sequence
  dRNA/arRNA
tgcattttgtaaaatagatactagcagattgtcccaagatgtgtacagctcattctcacagcccagcgagggcacctactccacaaatgcgtggccacaggtcatcacctgtcctgtggccctggcgagcctgatccctcacgccgggcac

SEQ ID NO: 160 - DNA, 151 bp, Artificial Sequence
  dRNA/arRNA
gctcattctcacagcccagcgagggcacttactccacaaatgcgtggccacaggtcatcacctgtcctgtggccccggcgagcctgatccctcacgccgggcacccacacggcctgcgtgccttctagacttgagttcgcagctctttaag

SEQ ID NO: 161 - DNA, 151 bp, Artificial Sequence
  dRNA/arRNA
tcggccgggccctgggggcggtgggcgctggccaggacgcccaccgtgtggttgctgtccaggacggtcccggcccgcgacacttcggcccagagctgctcctcatccagcagcgccagcagccccatggccgtgagcaccggcttgcgca

SEQ ID NO: 162 - RNA, 111 nt, Artificial Sequence
  dRNA/arRNA
ugaccagucuuaagaucuuucuugaccugcaccauaagaacuucuccaaagguaccaaaauacucuuucagguccuguucgguuguuuuccaugggagacccaacacuauu

SEQ ID NO: 163 - RNA, 111 nt, Artificial Sequence
  dRNA/arRNA
gaugggcaccaccccggugaacagcuccucgcccuugcucacuggcagagcccucgagcaucgcgagcaggcgcugccuccuccgcccugcagcuuguacagcucguccau

SEQ ID NO: 164 - RNA, 111 nt, Artificial Sequence
  dRNA/arRNA
gaugggcaccaccccggugaacagcuccucgcccuugcucacuggcagagcccuggagcaucgcgagcaggcgcugccuccuccgcccugcagcuuguacagcucguccau

SEQ ID NO: 165 - RNA, 111 nt, Artificial Sequence
  dRNA/arRNA
gaugggcaccaccccggugaacagcuccucgcccuugcucacuggcagagcccuugagcaucgcgagcaggcgcugccuccuccgcccugcagcuuguacagcucguccau

SEQ ID NO: 166 - RNA, 111 nt, Artificial Sequence
  dRNA/arRNA
gaugggcaccaccccggugaacagcuccucgcccuugcucacuggcagagcccuagagcaucgcgagcaggcgcugccuccuccgcccugcagcuuguacagcucguccau

SEQ ID NO: 167 - RNA, 111 nt, Artificial Sequence
  dRNA/arRNA
gaugggcaccaccccggugaacagcuccucgcccuugcucacuggcagagcccucgggcaucgcgagcaggcgcugccuccuccgcccugcagcuuguacagcucguccau

SEQ ID NO: 168 - RNA, 111 nt, Artificial Sequence
  dRNA/arRNA
gaugggcaccaccccggugaacagcuccucgcccuugcucacuggcagagcccuggggcaucgcgagcaggcgcugccuccuccgcccugcagcuuguacagcucguccau

SEQ ID NO: 169 - RNA, 111 nt, Artificial Sequence
  dRNA/arRNA
gaugggcaccaccccggugaacagcuccucgcccuugcucacuggcagagcccuugggcaucgcgagcaggcgcugccuccuccgcccugcagcuuguacagcucguccau

SEQ ID NO: 170 - RNA, 111 nt, Artificial Sequence
  dRNA/arRNA
gaugggcaccaccccggugaacagcuccucgcccuugcucacuggcagagcccuagggcaucgcgagcaggcgcugccuccuccgcccugcagcuuguacagcucguccau

SEQ ID NO: 171 - RNA, 111 nt, Artificial Sequence
  dRNA/arRNA
gaugggcaccaccccggugaacagcuccucgcccuugcucacuggcagagcccucgugcaucgcgagcaggcgcugccuccuccgcccugcagcuuguacagcucguccau

SEQ ID NO: 172 - RNA, 111 nt, Artificial Sequence
  dRNA/arRNA
gaugggcaccaccccggugaacagcuccucgcccuugcucacuggcagagcccuggugcaucgcgagcaggcgcugccuccuccgcccugcagcuuguacagcucguccau

SEQ ID NO: 173 - RNA, 111 nt, Artificial Sequence
  dRNA/arRNA
gaugggcaccaccccggugaacagcuccucgcccuugcucacuggcagagcccuagugcaucgcgagcaggcgcugccuccuccgcccugcagcuuguacagcucguccau

SEQ ID NO: 174 - RNA, 111 nt, Artificial Sequence
  dRNA/arRNA
gaugggcaccaccccggugaacagcuccucgcccuugcucacuggcagagcccuugugcaucgcgagcaggcgcugccuccuccgcccugcagcuuguacagcucguccau

SEQ ID NO: 175 - RNA, 111 nt, Artificial Sequence
  dRNA/arRNA
gaugggcaccaccccggugaacagcuccucgcccuugcucacuggcagagcccucgcgcaucgcgagcaggcgcugccuccuccgcccugcagcuuguacagcucguccau

SEQ ID NO: 176 - RNA, 111 nt, Artificial Sequence
  dRNA/arRNA
gaugggcaccaccccggugaacagcuccucgcccuugcucacuggcagagcccuggcgcaucgcgagcaggcgcugccuccuccgcccugcagcuuguacagcucguccau

SEQ ID NO: 177 - RNA, 111 nt, Artificial Sequence
  dRNA/arRNA
gaugggcaccaccccggugaacagcuccucgcccuugcucacuggcagagcccuugcgcaucgcgagcaggcgcugccuccuccgcccugcagcuuguacagcucguccau

SEQ ID NO: 178 - RNA, 111 nt, Artificial Sequence
  dRNA/arRNA
gaugggcaccaccccggugaacagcuccucgcccuugcucacuggcagagcccuagcgcaucgcgagcaggcgcugccuccuccgcccugcagcuuguacagcucguccau

SEQ ID NO: 179 - RNA, 111 nt, Artificial Sequence; identical to SEQ ID NO: 163
  dRNA/arRNA

SEQ ID NO: 180 - RNA, 111 nt, Artificial Sequence; identical to SEQ ID NO: 164
  dRNA/arRNA

SEQ ID NO: 181 - RNA, 111 nt, Artificial Sequence; identical to SEQ ID NO: 165
  dRNA/arRNA

SEQ ID NO: 182 - RNA, 111 nt, Artificial Sequence; identical to SEQ ID NO: 166
  dRNA/arRNA

SEQ ID NO: 183 - RNA, 111 nt, Artificial Sequence; identical to SEQ ID NO: 171
  dRNA/arRNA

SEQ ID NO: 184 - RNA, 111 nt, Artificial Sequence; identical to SEQ ID NO: 167
  dRNA/arRNA

SEQ ID NO: 185 - RNA, 111 nt, Artificial Sequence; identical to SEQ ID NO: 175
  dRNA/arRNA

SEQ ID NO: 186 - RNA, 111 nt, Artificial Sequence; identical to SEQ ID NO: 171
  dRNA/arRNA

SEQ ID NO: 187 - RNA, 111 nt, Artificial Sequence; identical to SEQ ID NO: 172
  dRNA/arRNA

SEQ ID NO: 188 - RNA, 111 nt, Artificial Sequence; identical to SEQ ID NO: 174
  dRNA/arRNA

SEQ ID NO: 189 - RNA, 111 nt, Artificial Sequence; identical to SEQ ID NO: 173
  dRNA/arRNA

SEQ ID NO: 190 - RNA, 111 nt, Artificial Sequence; identical to SEQ ID NO: 163
  dRNA/arRNA

SEQ ID NO: 191 - RNA, 111 nt, Artificial Sequence; identical to SEQ ID NO: 175
  dRNA/arRNA

SEQ ID NO: 192 - RNA, 111 nt, Artificial Sequence; identical to SEQ ID NO: 167
  dRNA/arRNA

SEQ ID NO: 193 - RNA, 111 nt, Artificial Sequence; identical to SEQ ID NO: 42
  dRNA/arRNA

SEQ ID NO: 194 - RNA, 111 nt, Artificial Sequence
  dRNA/arRNA
gauucugaauuagcuggaucgucaaggcacucgggccgacgccaccagcuccaaccaccacaaguggagagucagucauuuucagcaggccucucucccgcaccggggagc

SEQ ID NO: 195 - RNA, 111 nt, Artificial Sequence
  dRNA/arRNA
gggagcagccucuggcauucugggagcuucaucuggaccugggucuucagugaaccauuguucaauaucguccggggacagcaucaaaucauccauugcuugggacggcaa

SEQ ID NO: 196 - RNA, 111 nt, Artificial Sequence
  dRNA/arRNA
gggagcagccucuggcauucugggagcuucaucuggaccugggucuucagugaaccauuguucaagaucguccggggacagcaucaaaucauccauugcuugggacggcaa

SEQ ID NO: 197 - RNA, 111 nt, Artificial Sequence
  dRNA/arRNA
gggagcagccucuggcagucggggagcuucaucuggaccugggucuucagugaaccauuguucaagaucguccggggacagcaucaaaucauccagugcuugggacggcaa

SEQ ID NO: 198 - RNA, 111 nt, Artificial Sequence
  dRNA/arRNA
cauauuacagaauaccuugauagcauccaauuugcauccuugguuagggucaacccaguauucuccacucuugaguucaggauggcagaauuucaggucucugcaguuucu

SEQ ID NO: 199 - RNA, 111 nt, Artificial Sequence
  dRNA/arRNA
gugaagauaagccaguccucuaguaacagaaugagcaagacggcaagagcuuacccagucacuuguguggagacuuaaauacuugcauaaagauccauugggauaguacuc

SEQ ID NO: 200 - RNA, 111 nt, Artificial Sequence
  dRNA/arRNA
gugaacgucaaacugucggaccaauauggcagaaucuucucucaucucaacuuuccauauccguaucauggaaucauagcauccuguaacuacuagcucucuuacagcugg

SEQ ID NO: 201 - RNA, 111 nt, Artificial Sequence
  dRNA/arRNA
gccaaugaucucgugaguuaucucagcagugugagccaucagggugaugacaucccaggcgaucguguggccuccaggagcccagagcaggaaguugaggagaaggugccu

SEQ ID NO: 202 - RNA, 111 nt, Artificial Sequence
  dRNA/arRNA
caagacggugaaccacuccauggucuucuugucggcuuucugcacuguguacccccagagcuccguguugccgacauccugggguggcuuccacuccagagccacauuaag

SEQ ID NO: 203 - RNA, 111 nt, Artificial Sequence
  dRNA/arRNA
aggauucucuuuugaaguauugcucccccaguggauuggguggcuccauucacuccaaugcugagcacuuccacagaguggguuaaagcggcuccgaacacgaaacgugua

SEQ ID NO: 204 - RNA, 111 nt, Artificial Sequence
  dRNA/arRNA
gacgcccaccgugugguugcuguccaggacggucccggccugcgacacuucggcccagagcugcuccucauccagcagcgccagcagccccauggccgugagcaccggcuu

SEQ ID NO: 205 - RNA, 111 nt, Artificial Sequence
  dRNA/arRNA
gacgcccaccgugugguugcuguccaggacggucccggccugcgacacuucggcccagagcugcuccucaucugcggggcgggggggggccgucgccgcguggggucguug

SEQ ID NO: 206 - DNA, 31 bp, Artificial Sequence
  Primer
tataactagtatggtgagcaagggcgaggag

SEQ ID NO: 207 - DNA, 41 bp, Artificial Sequence
  Primer
tatacgtctcatctacagattcttccggcgtgtataccttc

SEQ ID NO: 208 - DNA, 53 bp, Artificial Sequence
  Primer
tatacgtctcatagagatccccggtcgccaccgtgagcaagggcgaggagctg

SEQ ID NO: 209 - DNA, 36 bp, Artificial Sequence
  Primer
tataggcgcgccttacttgtacagctcgtccatgcc

SEQ ID NO: 210 - DNA, 94 bp, Artificial Sequence
  Primer
tatacgtctcaaggcgctgcctcctccgccgctgcctcctccgccgctgcctcctccgccctgcagcttgtacagctcgtccatgccgccggtg

SEQ ID NO: 211 - DNA, 62 bp, Artificial Sequence
  Primer
tatacgtctcagcctgctcgcgatgctagagggctctgccagtgagcaagggcgaggagctg

SEQ ID NO: 212 - DNA, 70 bp, Artificial Sequence
  Primer
tataactagtatggtggattacaaggatgacgacgataagatgaaagtgacgaaggtaggaggcatttcg

SEQ ID NO: 213 - DNA, 60 bp, Artificial Sequence
  Primer
atatggcgcgccgttttcagactttttctcttccattttgtattcaaacataatcttcac

SEQ ID NO: 214 - DNA, 69 bp, Artificial Sequence
  Primer
tataggcgcgccaggcggaggaggcagcggcggaggaggcagcctcctcctctcaaggtccccagaagc

SEQ ID NO: 215 - DNA, 64 bp, Artificial Sequence
  Primer
tatacctgcaggctacaccttgcgttttttcttgggtactgggcagagataaaagttcttttcc

SEQ ID NO: 216 - DNA, 24 bp, Artificial Sequence
  Primer
cactccaccggcggcatggacgag

SEQ ID NO: 217 - DNA, 28 bp, Artificial Sequence
  Primer
cacgctgaacttgtggccgtttacgtcg

SEQ ID NO: 218 - DNA, 40 bp, Artificial Sequence
  Primer
tataactagtatgaatccgcggcaggggtattccctcagc

SEQ ID NO: 219 - DNA, 73 bp, Artificial Sequence
  Primer
tataggcgcgccctacttatcgtcgtcatccttgtaatctactgggcagagataaaagttcttttcctcctgg

SEQ ID NO: 220 - DNA, 42 bp, Artificial Sequence
  Primer
tataactagtatggatatagaagatgaagaaaacatgagttc

SEQ ID NO: 221 - DNA, 67 bp, Artificial Sequence
  Primer
tataggcgcgccctacttatcgtcgtcatccttgtaatcgggcgtgagtgagaactggtcctgctcg

SEQ ID NO: 222 - DNA, 37 bp, Artificial Sequence
  Primer
tataactagtatggccgagatcaaggagaaaatctgc

SEQ ID NO: 223 - DNA, 73 bp, Artificial Sequence; identical to SEQ ID NO: 219
  Primer

SEQ ID NO: 224 - DNA, 19 bp, Artificial Sequence
  Primer
cgccatttcggactgggag

SEQ ID NO: 225 - DNA, 25 bp, Artificial Sequence
  Primer
agagacaggtttctccatcaattac

SEQ ID NO: 226 - DNA, 16 bp, Artificial Sequence
  Primer
gagcccgcgagcaacc

SEQ ID NO: 227 - DNA, 20 bp, Artificial Sequence
  Primer
gcagcaggaagaagacggac

SEQ ID NO: 228 - DNA, 23 bp, Artificial Sequence
  Primer
agaagcagttgaagaccagactc

SEQ ID NO: 229 - DNA, 20 bp, Artificial Sequence
  Primer
ggccttcacctggaccatag

SEQ ID NO: 230 - DNA, 22 bp, Artificial Sequence
  Primer
agagaagcagttgaagaccaga

SEQ ID NO: 231 - DNA, 20 bp, Artificial Sequence
  Primer
cggccttcacctggaccata

SEQ ID NO: 232 - DNA, 23 bp, Artificial Sequence
  Primer
cagagaagcagttgaagaccaga

SEQ ID NO: 233 - DNA, 20 bp, Artificial Sequence
  Primer
cggccttcacctggaccata

SEQ ID NO: 234 - DNA, 20 bp, Artificial Sequence
  Primer
tttgtgaaaggctggggacc

SEQ ID NO: 235 - DNA, 25 bp, Artificial Sequence
  Primer
acaggattgtattttgtagtccacc

SEQ ID NO: 236 - DNA, 23 bp, Artificial Sequence
  Primer
aggatgagttttgtgaaaggctg

SEQ ID NO: 237 - DNA, 24 bp, Artificial Sequence
  Primer
attttgtagtccaccatcctgata

SEQ ID NO: 238 - DNA, 22 bp, Artificial Sequence
  Primer
gatgagttttgtgaaaggctgg

SEQ ID NO: 239 - DNA, 25 bp, Artificial Sequence
  Primer
attttgtagtccaccatcctgataa

SEQ ID NO: 240 - DNA, 20 bp, Artificial Sequence
  Primer
cgaagagaacgagaccgcat

SEQ ID NO: 241 - DNA, 19 bp, Artificial Sequence
  Primer
gaagatggtgcacaccggg

SEQ ID NO: 242 - DNA, 22 bp, Artificial Sequence
  Primer
gacagatgcttcatcagcagtg

SEQ ID NO: 243 - DNA, 21 bp, Artificial Sequence
  Primer
cgaacaaagccaaaccccttt

SEQ ID NO: 244 - DNA, 25 bp, Artificial Sequence
  Primer
tctgttaatggacaaatagaaagcc

SEQ ID NO: 245 - DNA, 23 bp, Artificial Sequence
  Primer
ggaacattcaaaggattggcact

SEQ ID NO: 246 - DNA, 20 bp, Artificial Sequence
  Primer
agtcactgcagatggacgca

SEQ ID NO: 247 - DNA, 22 bp, Artificial Sequence
  Primer
atctcgatgggaaattgcaggt

SEQ ID NO: 248 - DNA, 25 bp, Artificial Sequence
  Primer
tcagagttttacctcatccttcttt

SEQ ID NO: 249 - DNA, 25 bp, Artificial Sequence
  Primer
cctgaatacatatgatgaccttcag

SEQ ID NO: 250 - DNA, 20 bp, Artificial Sequence
  Primer
agggcacagacacagacctc

SEQ ID NO: 251 - DNA, 21 bp, Artificial Sequence
  Primer
agggctttcaatgccaagacg

SEQ ID NO: 252 - DNA, 19 bp, Artificial Sequence
  Primer
tgacaagccaagtcctccc

SEQ ID NO: 253 - DNA, 21 bp, Artificial Sequence
  Primer
attgccaatgatgagctctgg

SEQ ID NO: 254 - DNA, 25 bp, Artificial Sequence
  Primer
ttatagacataagttctccttgcct

SEQ ID NO: 255 - DNA, 20 bp, Artificial Sequence
  Primer
tcaatcccatggagccaaca

SEQ ID NO: 256 - DNA, 50 bp, Artificial Sequence
  Primer
tacacgacgctcttccgatcttaagtagaggccgccactccaccggcggc

SEQ ID NO: 257 - DNA, 51 bp, Artificial Sequence
  Primer
tacacgacgctcttccgatctatcatgcttagccgccactccaccggcggc

SEQ ID NO: 258 - DNA, 52 bp, Artificial Sequence
  dRNA/arRNA
tacacgacgctcttccgatctgatgcacatctgccgccactccaccggcggc

SEQ ID NO: 259 - DNA, 53 bp, Artificial Sequence
  Primer
tacacgacgctcttccgatctcgattgctcgacgccgccactccaccggcggc

SEQ ID NO: 260 - DNA, 54 bp, Artificial Sequence
  Primer
tacacgacgctcttccgatcttcgatagcaattcgccgccactccaccggcggc

SEQ ID NO: 261 - DNA, 55 bp, Artificial Sequence
  Primer
tacacgacgctcttccgatctatcgatagttgcttgccgccactccaccggcggc

SEQ ID NO: 262 - DNA, 56 bp, Artificial Sequence
  Primer
tacacgacgctcttccgatctgatcgatccagttaggccgccactccaccggcggc

SEQ ID NO: 263 - DNA, 57 bp, Artificial Sequence
  Primer
tacacgacgctcttccgatctcgatcgatttgagcctgccgccactccaccggcggc

SEQ ID NO: 264 - DNA, 58 bp, Artificial Sequence
  Primer
tacacgacgctcttccgatctacgatcgatacacgatcgccgccactccaccggcggc

SEQ ID NO: 265 - DNA, 59 bp, Artificial Sequence
  Primer
tacacgacgctcttccgatcttacgatcgatggtccagagccgccactccaccggcggc

SEQ ID NO: 266 - DNA, 50 bp, Artificial Sequence
  Primer
agacgtgtgctcttccgatcttaagtagagtcgccgtccagctcgaccag

SEQ ID NO: 267 - DNA, 51 bp, Artificial Sequence
  Primer
agacgtgtgctcttccgatctatcatgcttatcgccgtccagctcgaccag

SEQ ID NO: 268 - DNA, 52 bp, Artificial Sequence
  Primer
agacgtgtgctcttccgatctgatgcacatcttcgccgtccagctcgaccag

SEQ ID NO: 269 - DNA, 53 bp, Artificial Sequence
  Primer
agacgtgtgctcttccgatctcgattgctcgactcgccgtccagctcgaccag

SEQ ID NO: 270 - DNA, 54 bp, Artificial Sequence
  Primer
agacgtgtgctcttccgatcttcgatagcaattctcgccgtccagctcgaccag

SEQ ID NO: 271 - DNA, 55 bp, Artificial Sequence
  Primer
agacgtgtgctcttccgatctatcgatagttgctttcgccgtccagctcgaccag

SEQ ID NO: 272 - DNA, 56 bp, Artificial Sequence
  Primer
agacgtgtgctcttccgatctgatcgatccagttagtcgccgtccagctcgaccag

SEQ ID NO: 273 - DNA, 57 bp, Artificial Sequence
  Primer
agacgtgtgctcttccgatctcgatcgatttgagccttcgccgtccagctcgaccag

SEQ ID NO: 274 - DNA, 58 bp, Artificial Sequence
  Primer
agacgtgtgctcttccgatctacgatcgatacacgatctcgccgtccagctcgaccag

SEQ ID NO: 275 - DNA, 59 bp, Artificial Sequence
  Primer
agacgtgtgctcttccgatcttacgatcgatggtccagatcgccgtccagctcgaccag

SEQ ID NO: 276 - DNA, 18 bp, Artificial Sequence
  Primer
ggggaactcgggcaacct

SEQ ID NO: 277 - DNA, 19 bp, Artificial Sequence
  Primer
gaatcggatctgccccgtg

SEQ ID NO: 278 - DNA, 19 bp, Artificial Sequence
  Primer
catcgaggccaagctggaa

SEQ ID NO: 279 - DNA, 20 bp, Artificial Sequence
  Primer
gtagtgaggagggagacccc

SEQ ID NO: 280 - DNA, 20 bp, Artificial Sequence
  Primer
aagcctccttccttccccaa

SEQ ID NO: 281 - DNA, 21 bp, Artificial Sequence
  Primer
atcgatacactccctagccca

SEQ ID NO: 282 - DNA, 22 bp, Artificial Sequence
  Primer
acaaattcggtacatcctcgac

SEQ ID NO: 283 - DNA, 21 bp, Artificial Sequence
  Primer
ttcagccatctttggaaggtt

SEQ ID NO: 284 - DNA, 20 bp, Artificial Sequence
  Primer
acgccgcattgaccatctat

SEQ ID NO: 285 - DNA, 20 bp, Artificial Sequence
  Primer
tagccaggaggttctcaaca

SEQ ID NO: 286 - DNA, 21 bp, Artificial Sequence
  Primer
ggcatggactgtggtcatgag

SEQ ID NO: 287 - DNA, 20 bp, Artificial Sequence
  Primer
tgcaccaccaactgcttagc

SEQ ID NO: 288 - DNA, 22 bp, Artificial Sequence
  Primer
ccccgtaatgcagaagaagacc

SEQ ID NO: 289 - DNA, 21 bp, Artificial Sequence
  Primer
gtccttcagcttcagcctctg

SEQ ID NO: 290 - DNA, 20 bp, Artificial Sequence
  Primer
aacgcaacatgaaggtgctc

SEQ ID NO: 291 - DNA, 20 bp, Artificial Sequence
  Primer
accttgacggtgactttggg

SEQ ID NO: 292 - DNA, 20 bp, Artificial Sequence
  Primer
cagtgcaatgagggaccagt

SEQ ID NO: 293 - DNA, 24 bp, Artificial Sequence
  Primer
aggaccataggtacatcttcagag

SEQ ID NO: 294 - DNA, 22 bp, Artificial Sequence
  Primer
cgaacgagttgtatcacctgga

SEQ ID NO: 295 - DNA, 20 bp, Artificial Sequence
  Primer
cgatggctgtccctcaaagt

SEQ ID NO: 296 - DNA, 23 bp, Artificial Sequence
  Primer
agttgctcttttcactcaaggtc

SEQ ID NO: 297 - DNA, 21 bp, Artificial Sequence
  Primer
ttctctctgagttcagacgct

SEQ ID NO: 298 - DNA, 52 bp, Artificial Sequence
  Primer
tacacgacgctcttccgatcttaagtagagtggcacaggaggaaagagcatc

SEQ ID NO: 299 - DNA, 49 bp, Artificial Sequence
  Primer
agacgtgtgctcttccgatcttaagtagaggcaccacctccatgccctc

SEQ ID NO: 300 - DNA, 49 bp, Artificial Sequence
  Primer
tacacgacgctcttccgatcttaagtagagcatcgcagactgcggcaag

SEQ ID NO: 301 - DNA, 52 bp, Artificial Sequence
  Primer
agacgtgtgctcttccgatcttaagtagagagtccatgggcctgtggaatgt

SEQ ID NO: 302 - DNA, 19 bp, Artificial Sequence
  Primer
gaaaaactggcccgagagc

SEQ ID NO: 303 - DNA, 20 bp, Artificial Sequence
  Primer
ctgagtctgggctgagggac

SEQ ID NO: 304 - DNA, 20 bp, Artificial Sequence
  Primer
cgcttccaggtcaacaacac

SEQ ID NO: 305 - DNA, 19 bp, Artificial Sequence
  Primer
ctcgcgtagatcagcaccg

SEQ ID NO: 306 - DNA, 21 bp, Artificial Sequence
  Primer
cccctctgagtcaggaaacat

SEQ ID NO: 307 - DNA, 19 bp, Artificial Sequence
  Primer
gaagatgacaggggccagg

SEQ ID NO: 308 - DNA, 19 bp, Artificial Sequence
  Primer
tagcactggctggaatgag

SEQ ID NO: 309 - DNA, 21 bp, Artificial Sequence
  Primer
gtttcggaggtaacctgtaag

SEQ ID NO: 310 - DNA, 20 bp, Artificial Sequence
  Primer
tacagcaaccatgagtacaa

SEQ ID NO: 311 - DNA, 19 bp, Artificial Sequence
  Primer
tcaggtgtttcacataggc

SEQ ID NO: 312 - DNA, 19 bp, Artificial Sequence
  Primer
ctgcaaccatgagtgagaa

SEQ ID NO: 313 - DNA, 21 bp, Artificial Sequence
  Primer
cctttgaggtgctttagatag

SEQ ID NO: 314 - DNA, 19 bp, Artificial Sequence
  Primer
gccctgagaaaggagacat

SEQ ID NO: 315 - DNA, 24 bp, Artificial Sequence
  Primer
ctgttctggaggtactctaggtat

SEQ ID NO: 316 - DNA, 18 bp, Artificial Sequence
  Primer
tttgaagagggctgagaa

SEQ ID NO: 317 - DNA, 19 bp, Artificial Sequence
  Primer
tgttctggatatttcatgg

SEQ ID NO: 318 - DNA, 20 bp, Artificial Sequence
  Primer
catctgcctccccatattcc

SEQ ID NO: 319 - DNA, 22 bp, Artificial Sequence
  Primer
tccatcctagctcatctccaaa

SEQ ID NO: 320 - DNA, 18 bp, Artificial Sequence
  Primer
tgctccagaaggccagac

SEQ ID NO: 321 - DNA, 25 bp, Artificial Sequence
  Primer
ttcataaatactactaaggcacagg

SEQ ID NO: 322 - DNA, 21 bp, Artificial Sequence
  Primer
acagatgaagtgctccttcca

SEQ ID NO: 323 - DNA, 21 bp, Artificial Sequence
  Primer
gtcggagattcgtagctggat

SEQ ID NO: 324 - DNA, 21 bp, Artificial Sequence
  Primer
cattgtggccaaggagatctg

SEQ ID NO: 325 - DNA, 21 bp, Artificial Sequence
  Primer
cttcggagtttgggtttgctt

SEQ ID NO: 326 - DNA, 20 bp, Artificial Sequence
  Primer
catcacttgctgctgacacg

SEQ ID NO: 327 - DNA, 18 bp, Artificial Sequence
  dRNA/arRNA
tgtggaatctgccgggag

SEQ ID NO: 328 - DNA, 18 bp, Artificial Sequence
  Primer
ctgactctaagtggcatt

SEQ ID NO: 329 - DNA, 18 bp, Artificial Sequence
  dRNA/arRNA
tgatggccttcgattctg

SEQ ID NO: 330 - DNA, 23 bp, Artificial Sequence
  dRNA/arRNA
cggagtcaacggatttggtcgta

SEQ ID NO: 331 - DNA, 24 bp, Artificial Sequence
  Primer
agccttctccatggtggtgaagac

SEQ ID NO: 332 - DNA, 2820 bp, Artificial Sequence
  dRNA/arRNA
atggccgagatcaaggagaaaatctgcgactatctcttcaatgtgtctgactcctctgccctgaatttggctaaaaatattggccttaccaaggcccgagatataaatgctgtgctaattgacatggaaaggcagggggatgtctatagacaagggacaacccctcccatatggcatttgacagacaagaagcgagagaggatgcaaatcaagagaaatacgaacagtgttcctgaaaccgctccagctgcaatccctgagaccaaaagaaacgcagagttcctcacctgtaatatacccacatcaaatgcctcaaataacatggtaaccacagaaaaagtggagaatgggcaggaacctgtcataaagttagaaaacaggcaagaggccagaccagaaccagcaagactgaaaccacctgttcattacaatggcccctcaaaagcagggtatgttgactttgaaaatggccagtgggccacagatgacatcccagatgacttgaatagtatccgcgcagcaccaggtgagtttcgagccatcatggagatgccctccttctacagtcatggcttgccacggtgttcaccctacaagaaactgacagagtgccagctgaagaaccccatcagcgggctgttagaatatgcccagttcgctagtcaaacctgtgagttcaacatgatagagcagagtggaccaccccatgaacctcgatttaaattccaggttgtcatcaatggccgagagtttcccccagctgaagctggaagcaagaaagtggccaagcaggatgcagctatgaaagccatgacaattctgctagaggaagccaaagccaaggacagtggaaaatcagaagaatcatcccactattccacagagaaagaatcagagaagactgcagagtcccagacccccaccccttcagccacatccttcttttctgggaagagccccgtcaccacactgcttgagtgtatgcacaaattggggaactcctgcgaattccgtctcctgtccaaagaaggccctgcccatgaacccaagttccaatactgtgttgcagtgggagcccaaactttccccagtgtgagtgctcccagcaagaaagtggcaaagcagatggccgcagaggaagccatgaaggccctgcatggggaggcgaccaactccatggcttctgataaccagcctgaaggtatgatctcagagtcacttgataacttggaatccatgatgcccaacaaggtcaggaagattggcgagctcgtgagatacctgaacaccaaccctgtgggtggccttttggagtacgcccgctcccatggctttgctgctgaattcaagttggtcgaccagtccggacctcctcacgagcccaagttcgtttaccaagcaaaagttgggggtcgctggttcccagccgtctgcgcacacagcaagaagcaaggcaagcaggaagcagcagatgcggctctccgtgtcttgattggggagaacgagaaggcagaacgcatgggtttcacagaggtaaccccagtgacaggggccagtctcagaagaactatgctcctcctctcaaggtccccagaagcacagccaaagacactccctctcactggcagcaccttccatgaccagatagccatgctgagccaccggtgcttcaacactctgactaacagcttccagccctccttgctcggccgcaagattctggccgccatcattatgaaaaaagactctgaggacatgggtgtcgtcgtcagcttgggaacagggaatcgctgtgtaaaaggagattctctcagcctaaaaggagaaactgtcaatgactgccatgcagaaataatctcccggagaggcttcatcaggtttctctacagtgagttaatgaaatacaactcccagactgcgaaggatagtatatttgaacctgctaagggaggagaaaagctccaaataaaaaagactgtgtcattccatctgtatatcagcactgctccgtgtggagatggcgccctctttgacaagtcctgcagcgaccgtgctatggaaagcacagaatcccgccactaccctgtcttcgagaatcccaaacaaggaaagctccgcaccaaggtggagaacggagaaggcacaatccctgtggaatccagtgacattgtgcctacgtgggatggcattcggctcggggagagactccgtaccatgtcctgtagtgacaaaatcctacgctggaacgtgctgggcctgcaaggggcactgttgacccacttcctgcagcccatttatctcaaatctgtcacattgggttaccttttcagccaagggcatctgacccgtgctatttgctgtcgtgtgacaagagatgggagtgcatttgaggatggactacgacatccctttattgtcaaccaccccaaggttggcagagtcagcatatatgattccaaaaggcaatccgggaagactaaggagacaagcgtcaactggtgtctggctgatggctatgacctggagatcctggacggtaccagaggcactgtggatgggccacggaatgaattgtcccgggtctccaaaaagaacatttttcttctatttaagaagctctgctccttccgttaccgcagggatctactgagactctcctatggtgaggccaagaaagctgcccgtgactacgagacggccaagaactacttcaaaaaaggcctgaaggatatgggctatgggaactggattagcaaaccccaggaggaaaagaacttttatctctgcccagtagattacaaggatgacgacgataagtag

SEQ ID NO: 333 - DNA, 3705 bp, Artificial Sequence
  dRNA/arRNA
atgaatccgcggcaggggtattccctcagcggatactacacccatccatttcaaggctatgagcacagacagctcagataccagcagcctgggccaggatcttcccccagtagtttcctgcttaagcaaatagaatttctcaaggggcagctcccagaagcaccggtgattggaaagcagacaccgtcactgccaccttccctcccaggactccggccaaggtttccagtactacttgcctccagtaccagaggcaggcaagtggacatcaggggtgtccccaggggcgtgcatctcggaagtcaggggctccagagagggttccagcatccttcaccacgtggcaggagtctgccacagagaggtgttgattgcctttcctcacatttccaggaactgagtatctaccaagatcaggaacaaaggatcttaaagttcctggaagagcttggggaagggaaggccaccacagcacatgatctgtctgggaaacttgggactccgaagaaagaaatcaatcgagttttatactccctggcaaagaagggcaagctacagaaagaggcaggaacaccccctttgtggaaaatcgcggtctccactcaggcttggaaccagcacagcggagtggtaagaccagacggtcatagccaaggagccccaaactcagacccgagtttggaaccggaagacagaaactccacatctgtctcagaagatcttcttgagccttttattgcagtctcagctcaggcttggaaccagcacagcggagtggtaagaccagacagtcatagccaaggatccccaaactcagacccaggtttggaacctgaagacagcaactccacatctgccttggaagatcctcttgagtttttagacatggccgagatcaaggagaaaatctgcgactatctcttcaatgtgtctgactcctctgccctgaatttggctaaaaatattggccttaccaaggcccgagatataaatgctgtgctaattgacatggaaaggcagggggatgtctatagacaagggacaacccctcccatatggcatttgacagacaagaagcgagagaggatgcaaatcaagagaaatacgaacagtgttcctgaaaccgctccagctgcaatccctgagaccaaaagaaacgcagagttcctcacctgtaatatacccacatcaaatgcctcaaataacatggtaaccacagaaaaagtggagaatgggcaggaacctgtcataaagttagaaaacaggcaagaggccagaccagaaccagcaagactgaaaccacctgttcattacaatggcccctcaaaagcagggtatgttgactttgaaaatggccagtgggccacagatgacatcccagatgacttgaatagtatccgcgcagcaccaggtgagtttcgagccatcatggagatgccctccttctacagtcatggcttgccacggtgttcaccctacaagaaactgacagagtgccagctgaagaaccccatcagcgggctgttagaatatgcccagttcgctagtcaaacctgtgagttcaacatgatagagcagagtggaccaccccatgaacctcgatttaaattccaggttgtcatcaatggccgagagtttcccccagctgaagctggaagcaagaaagtggccaagcaggatgcagctatgaaagccatgacaattctgctagaggaagccaaagccaaggacagtggaaaatcagaagaatcatcccactattccacagagaaagaatcagagaagactgcagagtcccagacccccaccccttcagccacatccttcttttctgggaagagccccgtcaccacactgcttgagtgtatgcacaaattggggaactcctgcgaattccgtctcctgtccaaagaaggccctgcccatgaacccaagttccaatactgtgttgcagtgggagcccaaactttccccagtgtgagtgctcccagcaagaaagtggcaaagcagatggccgcagaggaagccatgaaggccctgcatggggaggcgaccaactccatggcttctgataaccagcctgaaggtatgatctcagagtcacttgataacttggaatccatgatgcccaacaaggtcaggaagattggcgagctcgtgagatacctgaacaccaaccctgtgggtggccttttggagtacgcccgctcccatggctttgctgctgaattcaagttggtcgaccagtccggacctcctcacgagcccaagttcgtttaccaagcaaaagttgggggtcgctggttcccagccgtctgcgcacacagcaagaagcaaggcaagcaggaagcagcagatgcggctctccgtgtcttgattggggagaacgagaaggcagaacgcatgggtttcacagaggtaaccccagtgacaggggccagtctcagaagaactatgctcctcctctcaaggtccccagaagcacagccaaagacactccctctcactggcagcaccttccatgaccagatagccatgctgagccaccggtgcttcaacactctgactaacagcttccagccctccttgctcggccgcaagattctggccgccatcattatgaaaaaagactctgaggacatgggtgtcgtcgtcagcttgggaacagggaatcgctgtgtaaaaggagattctctcagcctaaaaggagaaactgtcaatgactgccatgcagaaataatctcccggagaggcttcatcaggtttctctacagtgagttaatgaaatacaactcccagactgcgaaggatagtatatttgaacctgctaagggaggagaaaagctccaaataaaaaagactgtgtcattccatctgtatatcagcactgctccgtgtggagatggcgccctctttgacaagtcctgcagcgaccgtgctatggaaagcacagaatcccgccactaccctgtcttcgagaatcccaaacaaggaaagctccgcaccaaggtggagaacggagaaggcacaatccctgtggaatccagtgacattgtgcctacgtgggatggcattcggctcggggagagactccgtaccatgtcctgtagtgacaaaatcctacgctggaacgtgctgggcctgcaaggggcactgttgacccacttcctgcagcccatttatctcaaatctgtcacattgggttaccttttcagccaagggcatctgacccgtgctatttgctgtcgtgtgacaagagatgggagtgcatttgaggatggactacgacatccctttattgtcaaccaccccaaggttggcagagtcagcatatatgattccaaaaggcaatccgggaagactaaggagacaagcgtcaactggtgtctggctgatggctatgacctggagatcctggacggtaccagaggcactgtggatgggccacggaatgaattgtcccgggtctccaaaaagaacatttttcttctatttaagaagctctgctccttccgttaccgcagggatctactgagactctcctatggtgaggccaagaaagctgcccgtgactacgagacggccaagaactacttcaaaaaaggcctgaaggatatgggctatgggaactggattagcaaaccccaggaggaaaagaacttttatctctgcccagtagattacaaggatgacgacgataagtag

SEQ ID NO: 334 - DNA, 2130 bp, Artificial Sequence
  dRNA/arRNA
atggatatagaagatgaagaaaacatgagttccagcagcactgatgtgaaggaaaaccgcaatctggacaacgtgtcccccaaggatggcagcacacctgggcctggcgagggctctcagctctccaatgggggtggtggtggccccggcagaaagcggcccctggaggagggcagcaatggccactccaagtaccgcctgaagaaaaggaggaaaacaccagggcccgtcctccccaagaacgccctgatgcagctgaatgagatcaagcctggtttgcagtacacactcctgtcccagactgggcccgtgcacgcgcctttgtttgtcatgtctgtggaggtgaatggccaggtttttgagggctctggtcccacaaagaaaaaggcaaaactccatgctgctgagaaggccttgaggtctttcgttcagtttcctaatgcctctgaggcccacctggccatggggaggaccctgtctgtcaacacggacttcacatctgaccaggccgacttccctgacacgctcttcaatggttttgaaactcctgacaaggcggagcctcccttttacgtgggctccaatggggatgactccttcagttccagcggggacctcagcttgtctgcttccccggtgcctgccagcctagcccagcctcctctccctgccttaccaccattcccacccccgagtgggaagaatcccgtgatgatcttgaacgaactgcgcccaggactcaagtatgacttcctctccgagagcggggagagccatgccaagagcttcgtcatgtctgtggtcgtggatggtcagttctttgaaggctcggggagaaacaagaagcttgccaaggcccgggctgcgcagtctgccctggccgccatttttaacttgcacttggatcagacgccatctcgccagcctattcccagtgagggtcttcagctgcatttaccgcaggttttagctgacgctgtctcacgcctggtcctgggtaagtttggtgacctgaccgacaacttctcctcccctcacgctcgcagaaaagtgctggctggagtcgtcatgacaacaggcacagatgttaaagatgccaaggtgataagtgtttctacaggaacaaaatgtattaatggtgaatacatgagtgatcgtggccttgcattaaatgactgccatgcagaaataatatctcggagatccttgctcagatttctttatacacaacttgagctttacttaaataacaaagatgatcaaaaaagatccatctttcagaaatcagagcgaggggggtttaggctgaaggagaatgtccagtttcatctgtacatcagcacctctccctgtggagatgccagaatcttctcaccacatgagccaatcctggaagaaccagcagatagacacccaaatcgtaaagcaagaggacagctacggaccaaaatagagtctggtgaggggacgattccagtgcgctccaatgcgagcatccaaacgtgggacggggtgctgcaaggggagcggctgctcaccatgtcctgcagtgacaagattgcacgctggaacgtggtgggcatccagggatccctgctcagcattttcgtggagcccatttacttctcgagcatcatcctgggcagcctttaccacggggaccacctttccagggccatgtaccagcggatctccaacatagaggacctgccacctctctacaccctcaacaagcctttgctcagtggcatcagcaatgcagaagcacggcagccagggaaggcccccaacttcagtgtcaactggacggtaggcgactccgctattgaggtcatcaacgccacgactgggaaggatgagctgggccgcgcgtcccgcctgtgtaagcacgcgttgtactgtcgctggatgcgtgtgcacggcaaggttccctcccacttactacgctccaagattaccaaacccaacgtgtaccatgagtccaagctggcggcaaaggagtaccaggccgccaaggcgcgtctgttcacagccttcatcaaggcggggctgggggcctgggtggagaagcccaccgagcaggaccagttctcactcacgcccgattacaaggatgacgacgataagtag

SEQ ID NO: 335 - DNA, 4401 bp, Artificial Sequence
  dRNA/arRNA
atgatgagctttgtgcaaaaggggagctggctacttctcgctctgcttcatcccactattattttggcacaacaggaagctgttgaaggaggatgttcccatcttggtcagtcctatgcggatagagatgtctggaagccagaaccatgccaaatatgtgtctgtgactcaggatccgttctctgcgatgacataatatgtgacgatcaagaattagactgccccaacccagaaattccatttggagaatgttgtgcagtttgcccacagcctccaactgctcctactcgccctcctaatggtcaaggacctcaaggccccaagggagatccaggccctcctggtattcctgggagaaatggtgaccctggtattccaggacaaccagggtcccctggttctcctggcccccctggaatctgtgaatcatgccctactggtcctcagaactattctccccagtatgattcatatgatgtcaagtctggagtagcagtaggaggactcgcaggctatcctggaccagctggccccccaggccctcccggtccccctggtacatctggtcatcctggttcccctggatctccaggataccaaggaccccctggtgaacctgggcaagctggtccttcaggccctccaggacctcctggtgctataggtccatctggtcctgctggaaaagatggagaatcaggtagacccggacgacctggagagcgaggattgcctggacctccaggtatcaaaggtccagctgggatacctggattccctggtatgaaaggacacagaggcttcgatggacgaaatggagaaaagggtgaaacaggtgctcctggattaaagggtgaaaatggtcttccaggcgaaaatggagctcctggacccatgggtccaagaggggctcctggtgagcgaggacggccaggacttcctggggctgcaggtgctcggggtaatgacggtgctcgaggcagtgatggtcaaccaggccctcctggtcctcctggaactgccggattccctggatcccctggtgctaagggtgaagttggacctgcagggtctcctggttcaaatggtgcccctggacaaagaggagaacctggacctcagggacacgctggtgctcaaggtcctcctggccctcctgggattaatggtagtcctggtggtaaaggcgaaatgggtcccgctggcattcctggagctcctggactgatgggagcccggggtcctccaggaccagccggtgctaatggtgctcctggactgcgaggtggtgcaggtgagcctggtaagaatggtgccaaaggagagcccggaccacgtggtgaacgcggtgaggctggtattccaggtgttccaggagctaaaggcgaagatggcaaggatggatcacctggagaacctggtgcaaatgggcttccaggagctgcaggagaaaggggtgcccctgggttccgaggacctgctggaccaaatggcatcccaggagaaaagggtcctgctggagagcgtggtgctccaggccctgcagggcccagaggagctgctggagaacctggcagagatggcgtccctggaggtccaggaatgaggggcatgcccggaagtccaggaggaccaggaagtgatgggaaaccagggcctcccggaagtcaaggagaaagtggtcgaccaggtcctcctgggccatctggtccccgaggtcagcctggtgtcatgggcttccccggtcctaaaggaaatgatggtgctcctggtaagaatggagaacgaggtggccctggaggacctggccctcagggtcctcctggaaagaatggtgaaactggacctcagggacccccagggcctactgggcctggtggtgacaaaggagacacaggaccccctggtccacaaggattacaaggcttgcctggtacaggtggtcctccaggagaaaatggaaaacctggggaaccaggtccaaagggtgatgccggtgcacctggagctccaggaggcaagggtgatgctggtgcccctggtgaacgtggacctcctggattggcaggggccccaggacttagaggtggagctggtccccctggtcccgaaggaggaaagggtgctgctggtcctcctgggccacctggtgctgctggtactcctggtctgcaaggaatgcctggagaaagaggaggtcttggaagtcctggtccaaagggtgacaagggtgaaccaggcggtccaggtgctgatggtgtcccagggaaagatggcccaaggggtcctactggtcctattggtcctcctggcccagctggccagcctggagataagggtgaaggtggtgcccccggacttccaggtatagctggacctcgtggtagccctggtgagagaggtgaaactggccctccaggacctgctggtttccctggtgctcctggacagaatggtgaacctggtggtaaaggagaaagaggggctccgggtgagaaaggtgaaggaggccctcctggagttgcaggaccccctggaggttctggacctgctggtcctcctggtccccaaggtgtcaaaggtgaacgtggcagtcctggtggacctggtgctgctggcttccctggtgctcgtggtcttcctggtcctcctggtagtaatggtaacccaggacccccaggtcccagcggttctccaggcaaggatgggcccccaggtcctgcgggtaacactggtgctcctggcagccctggagtgtctggaccaaaaggtgatgctggccaaccaggagagaagggatcgcctggtgcccagggcccaccaggagctccaggcccacttgggattgctgggatcactggagcacggggtcttgcaggaccaccaggcatgccaggtcctaggggaagccctggccctcagggtgtcaagggtgaaagtgggaaaccaggagctaacggtctcagtggagaacgtggtccccctggaccccagggtcttcctggtctggctggtacagctggtgaacctggaagagatggaaaccctggatcagatggtcttccaggccgagatggatctcctggtggcaagggtgatcgtggtgaaaatggctctcctggtgcccctggcgctcctggtcatccaggcccacctggtcctgtcggtccagctggaaagagtggtgacagaggagaaagtggccctgctggccctgctggtgctcccggtcctgctggttcccgaggtgctcctggtcctcaaggcccacgtggtgacaaaggtgaaacaggtgaacgtggagctgctggcatcaaaggacatcgaggattccctggtaatccaggtgccccaggttctccaggccctgctggtcagcagggtgcaatcggcagtccaggacctgcaggccccagaggacctgttggacccagtggacctcctggcaaagatggaaccagtggacatccaggtcccattggaccaccagggcctcgaggtaacagaggtgaaagaggatctgagggctccccaggccacccagggcaaccaggccctcctggacctcctggtgcccctggtccttgctgtggtggtgttggagccgctgccattgctgggattggaggtgaaaaagctggcggttttgccccgtattatggagatgaaccaatggatttcaaaatcaacaccgatgagattatgacttcactcaagtctgttaatggacaaatagaaagcctcattagtcctgatggttctcgtaaaaaccccgctagaaactgcagagacctgaaattctgccatcctgaactcaagagtggagaatactgggttgaccctaaccaaggatgcaaattggatgctatcaaggtattctgtaatatggaaactggggaaacatgcataagtgccaatcctttgaatgttccacggaaacactggtggacagattctagtgctgagaagaaacacgtttggtttggagagtccatggatggtggttttcagtttagctacggcaatcctgaacttcctgaagatgtccttgatgtgcagctggcattccttcgacttctctccagccgagcttcccagaacatcacatatcactgcaaaaatagcattgcatacatggatcaggccagtggaaatgtaaagaaggccctgaagctgatggggtcaaatgaaggtgaattcaaggctgaaggaaatagcaaattcacctacacagttctggaggatggttgcacgaaacacactggggaatggagcaaaacagtctttgaatatcgaacacgcaaggctgtgagactacctattgtagatattgcaccctatgacattggtggtcctgatcaagaatttggtgtggacgttggccctgtttgctttttataa

SEQ ID NO: 336 - DNA, 3117 bp, Artificial Sequence
  dRNA/arRNA
atgacttcctcgctgcagcggccctggcgggtgccctggctaccatggaccatcctgctggtcagcgctgcggctgcttcgcagaatcaagaacggctatgtgcgtttaaagatccgtatcagcaagaccttgggataggtgagagtagaatctctcatgaaaatgggacaatattatgctcgaaaggtagcacctgctatggcctttgggagaaatcaaaaggggacataaatcttgtaaaacaaggatgttggtctcacattggagatccccaagagtgtcactatgaagaatgtgtagtaactaccactcctccctcaattcagaatggaacataccgtttctgctgttgtagcacagatttatgtaatgtcaactttactgagaattttccacctcctgacacaacaccactcagtccacctcattcatttaaccgagatgagacaataatcattgctttggcatcagtctctgtattagctgttttgatagttgccttatgctttggatacagaatgttgacaggagaccgtaaacaaggtcttcacagtatgaacatgatggaggcagcagcatccgaaccctctcttgatctagataatctgaaactgttggagctgattggccgaggtcgatatggagcagtatataaaggctccttggatgagcgtccagttgctgtaaaagtgttttcctttgcaaaccgtcagaattttatcaacgaaaagaacatttacagagtgcctttgatggaacatgacaacattgcccgctttatagttggagatgagagagtcactgcagatggacgcatggaatatttgcttgtgatggagtactatcccaatggatctttatgcaagtatttaagtctccacacaagtgactgggtaagctcttgccgtcttgctcattctgttactagaggactggcttatcttcacacagaattaccacgaggagatcattataaacctgcaatttcccatcgagatttaaacagcagaaatgtcctagtgaaaaatgatggaacctgtgttattagtgactttggactgtccatgaggctgactggaaatagactggtgcgcccaggggaggaagataatgcagccataagcgaggttggcactatcagatatatggcaccagaagtgctagaaggagctgtgaacttgagggactgtgaatcagctttgaaacaagtagacatgtatgctcttggactaatctattgggagatatttatgagatgtacagacctcttcccaggggaatccgtaccagagtaccagatggcttttcagacagaggttggaaaccatcccacttttgaggatatgcaggttctcgtgtctagggaaaaacagagacccaagttcccagaagcctggaaagaaaatagcctggcagtgaggtcactcaaggagacaatcgaagactgttgggaccaggatgcagaggctcggcttactgcacagtgtgctgaggaaaggatggctgaacttatgatgatttgggaaagaaacaaatctgtgagcccaacagtcaatccaatgtctactgctatgcagaatgaacgcaacctgtcacataataggcgtgtgccaaaaattggtccttatccagattattcttcctcctcatacattgaagactctatccatcatactgacagcatcgtgaagaatatttcctctgagcattctatgtccagcacacctttgactataggggaaaaaaaccgaaattcaattaactatgaacgacagcaagcacaagctcgaatccccagccctgaaacaagtgtcaccagcctctccaccaacacaacaaccacaaacaccacaggactcacgccaagtactggcatgactactatatctgagatgccatacccagatgaaacaaatctgcataccacaaatgttgcacagtcaattgggccaacccctgtctgcttacagctgacagaagaagacttggaaaccaacaagctagacccaaaagaagttgataagaacctcaaggaaagctctgatgagaatctcatggagcactctcttaaacagttcagtggcccagacccactgagcagtactagttctagcttgctttacccactcataaaacttgcagtagaagcaactggacagcaggacttcacacagactgcaaatggccaagcatgtttgattcctgatgttctgcctactcagatctatcctctccccaagcagcagaaccttcccaagagacctactagtttgcctttgaacaccaaaaattcaacaaaagagccccggctaaaatttggcagcaagcacaaatcaaacttgaaacaagtcgaaactggagttgccaagatgaatacaatcaatgcagcagaacctcatgtggtgacagtcaccatgaatggtgtggcaggtagaaaccacagtgttaactcccatgctgccacaacccaatatgccaatgggacagtactatctggccaaacaaccaacatagtgacacatagggcccaagaaatgttgcagaatcagtttattggtgaggacacccggctgaatattaattccagtcctgatgagcatgagcctttactgagacgagagcaacaagctggccatgatgaaggtgttctggatcgtcttgtggacaggagggaacggccactagaaggtggccgaactaattccaataacaacaacagcaatccatgttcagaacaagatgttcttgcacagggtgttccaagcacagcagcagatcctgggccatcaaagcccagaagagcacagaggcctaattctctggatctttcagccacaaatgtcctggatggcagcagtatacagataggtgagtcaacacaagatggcaaatcaggatcaggtgaaaagatcaagaaacgtgtgaaaactccctattctcttaagcggtggcgcccctccacctgggtcatctccactgaatcgctggactgtgaagtcaacaataatggcagtaacagggcagttcattccaaatccagcactgctgtttaccttgcagaaggaggcactgctacaaccatggtgtctaaagatataggaatgaactgtctgtga

SEQ ID NO: 337 - DNA, 3590 bp, Artificial Sequence
  dRNA/arRNA
atgcctacagctgagagtgaagcaaaagtaaaaaccaaagttcgctttgaagaattgcttaagacccacagtgatctaatgcgtgaaaagaaaaaactgaagaaaaaacttgtcaggtctgaagaaaacatctcacctgacactattagaagcaatcttcactatatgaaagaaactacaagtgatgatcccgacactattagaagcaatcttccccatattaaagaaactacaagtgatgatgtaagtgctgctaacactaacaacctgaagaagagcacgagagtcactaaaaacaaattgaggaacacacagttagcaactgaaaatcctaatggtgatgctagtgtagaggaagacaaacaaggaaagccaaataaaaaggtgataaagacggtgccccagttgactacacaagacctgaaaccggaaactcctgagaataaggttgattctacacaccagaaaacacatacaaagccacagccaggcgttgatcatcagaaaagtgagaaggcaaatgagggaagagaagagactgatttagaagaggatgaagaattgatgcaagcatatcagtgccatgtaactgaagaaatggcaaaggagattaagaggaaaataagaaagaaactgaaagaacagttgacttactttccctcagatactttattccatgatgacaaactaagcagtgaaaaaaggaaaaagaaaaaggaagttccagtcttctctaaagctgaaacaagtacattgaccatctctggtgacacagttgaaggtgaacaaaagaaagaatcttcagttagatcagtttcttcagattctcatcaagatgatgaaataagctcaatggaacaaagcacagaagacagcatgcaagatgatacaaaacctaaaccaaaaaaaacaaaaaagaagactaaagcagttgcagataataatgaagatgttgatggtgatggtgttcatgaaataacaagccgagatagcccggtttatcccaaatgtttgcttgatgatgaccttgtcttgggagtttacattcaccgaactgatagacttaagtcagattttatgatttctcacccaatggtaaaaattcatgtggttgatgagcatactggtcaatatgtcaagaaagatgatagtggacggcctgtttcatcttactatgaaaaagagaatgtggattatattcttcctattatgacccagccatatgattttaaacagttaaaatcaagacttccagagtgggaagaacaaattgtatttaatgaaaattttccctatttgcttcgaggctctgatgagagtcctaaagtcatcctgttctttgagattcttgatttcttaagcgtggatgaaattaagaataattctgaggttcaaaaccaagaatgtggctttcggaaaattgcctgggcatttcttaagcttctgggagccaatggaaatgcaaacatcaactcaaaacttcgcttgcagctatattacccacctactaagcctcgatccccattaagtgttgttgaggcatttgaatggtggtcaaaatgtccaagaaatcattacccatcaacactgtacgtaactgtaagaggactgaaagttccagactgtataaagccatcttaccgctctatgatggctcttcaggaggaaaaaggtaaaccagtgcattgtgaacgtcaccatgagtcaagctcagtagacacagaacctggattagaagagtcaaaggaagtaataaagtggaaacgactccctgggcaggcttgccgtatcccaaacaaacacctcttctcactaaatgcaggagaacgaggatgtttttgtcttgatttctcccacaatggaagaatattagcagcagcttgtgccagccgggatggatatccaattattttatatgaaattccttctggacgtttcatgagagaattgtgtggccacctcaatatcatttatgatctttcctggtcaaaagatgatcactacatccttacttcatcatctgatggcactgccaggatatggaaaaatgaaataaacaatacaaatactttcagagttttacctcatccttcttttgtttacacggctaaattccatccagctgtaagagagctagtagttacaggatgctatgattccatgatacggatatggaaagttgagatgagagaagattctgccatattggtccgacagtttgacgttcacaaaagttttatcaactcactttgttttgatactgaaggtcatcatatgtattcaggagattgtacaggggtgattgttgtttggaatacctatgtcaagattaatgatttggaacattcagtgcaccactggactataaataaggaaattaaagaaactgagtttaagggaattccaataagttatttggagattcatcccaatggaaaacgtttgttaatccataccaaagacagtactttgagaattatggatctccggatattagtagcaaggaagtttgtaggagcagcaaattatcgggagaagattcatagtactttgactccatgtgggacttttctgtttgctggaagtgaggatggtatagtgtatgtttggaacccagaaacaggagaacaagtagccatgtattctgacttgccattcaagtcacccattcgagacatttcttatcatccatttgaaaatatggttgcattctgtgcatttgggcaaaatgagccaattcttctgtatatttacgatttccatgttgcccagcaggaggctgaaatgttcaaacgctacaatggaacatttccattacctggaatacaccaaagtcaagatgccctatgtacctgtccaaaactaccccatcaaggctcttttcagattgatgaatttgtccacactgaaagttcttcaacgaagatgcagctagtaaaacagaggcttgaaactgtcacagaggtgatacgttcctgtgctgcaaaagtcaacaaaaatctctcatttacttcaccaccagcagtttcctcacaacagtctaagttaaagcagtcaaacatgctgaccgctcaagagattctacatcagtttggtttcactcagaccgggattatcagcatagaaagaaagccttgtaaccatcaggtagatacagcaccaacggtagtggctctttatgactacacagcgaatcgatcagatgaactaaccatccatcgcggagacattatccgagtgtttttcaaagataatgaagactggtggtatggcagcataggaaagggacaggaaggttattttccagctaatcatgtggctagtgaaacactgtatcaagaactgcctcctgagataaaggagcgatcccctcctttaagccctgaggaaaaaactaaaatagaaaaatctccagctcctcaaaagcaatcaatcaataagaacaagtcccaggacttcagactaggctcagaatctatgacacattctgaaatgagaaaagaacagagccatgaggaccaaggacacataatggatacacggatgaggaagaacaagcaagcaggcagaaaagtcactctaatagagta

SEQ ID NO: 338 - DNA, 1677 bp, Artificial Sequence
  dRNA/arRNA
atggctcaagattcagtagatctttcttgtgattatcagttttggatgcagaagctttctgtatgggatcaggcttccactttggaaacccagcaagacacctgtcttcacgtggctcagttccaggagttcctaaggaagatgtatgaagccttgaaagagatggattctaatacagtcattgaaagattccccacaattggtcaactgttggcaaaagcttgttggaatccttttattttagcatatgatgaaagccaaaaaattctaatatggtgcttatgttgtctaattaacaaagaaccacagaattctggacaatcaaaacttaactcctggatacagggtgtattatctcatatactttcagcactcagatttgataaagaagttgctcttttcactcaaggtcttgggtatgcacctatagattactatcctggtttgcttaaaaatatggttttatcattagcgtctgaactcagagagaatcatcttaatggatttaacactcaaaggcgaatggctcccgagcgagtggcgtccctgtcacgagtttgtgtcccacttattaccctgacagatgttgaccccctggtggaggctctcctcatctgtcatggacgtgaacctcaggaaatcctccagccagagttctttgaggctgtaaacgaggccattttgctgaagaagatttctctccccatgtcagctgtagtctgcctctggcttcggcaccttcccagccttgaaaaagcaatgctgcatctttttgaaaagctaatctccagtgagagaaattgtctgagaaggatcgaatgctttataaaagattcatcgctgcctcaagcagcctgccaccctgccatattccgggttgttgatgagatgttcaggtgtgcactcctggaaaccgatggggccctggaaatcatagccactattcaggtgtttacgcagtgctttgtagaagctctggagaaagcaagcaagcagctgcggtttgcactcaagacctactttccttacacttctccatctcttgccatggtgctgctgcaagaccctcaagatatccctcggggacactggctccagacactgaagcatatttctgaactgctcagagaagcagttgaagaccagactcatgggtcctgcggaggtccctttgagagctggttcctgttcattcacttcggaggatgggctgagatggtggcagagcaattactgatgtcggcagccgaaccccccacggccctgctgtggctcttggccttctactacggcccccgtgatgggaggcagcagagagcacagactatggtccaggtgaaggccgtgctgggccacctcctggcaatgtccagaagcagcagcctctcagcccaggacctgcagacggtagcaggacagggcacagacacagacctcagagctcctgcacaacagctgatcaggcaccttctcctcaacttcctgctctgggctcctggaggccacacgatcgcctgggatgtcatcaccctgatggctcacactgctgagataactcacgagatcattggctttcttgaccagaccttgtacagatggaatcgtcttggcattgaaagccctagatcagaaaaactggcccgagagctccttaaagagctgcgaactcaagtctag

SEQ ID NO: 339 - DNA, 3825 bp, Artificial Sequence
  dRNA/arRNA
atgcctgagccggggaagaagccagtctcagcttttagcaagaagccacggtcagtggaagtggccgcaggcagccctgccgtgttcgaggccgagacagagcgggcaggagtgaaggtgcgctggcagcgcggaggcagtgacatcagcgccagcaacaagtacggcctggccacagagggcacacggcatacgctgacagtgcgggaagtgggccctgccgaccagggatcttacgcagtcattgctggctcctccaaggtcaagttcgacctcaaggtcatagaggcagagaaggcagagcccatgctggcccctgcccctgcccctgctgaggccactggagcccctggagaagccccggccccagccgctgagctgggagaaagtgccccaagtcccaaagggtcaagctcagcagctctcaatggtcctacccctggagcccccgatgaccccattggcctcttcgtgatgcggccacaggatggcgaggtgaccgtgggtggcagcatcaccttctcagcccgcgtggccggcgccagcctcctgaagccgcctgtggtcaagtggttcaagggcaaatgggtggacctgagcagcaaggtgggccagcacctgcagctgcacgacagctacgaccgcgccagcaaggtctatctgttcgagctgcacatcaccgatgcccagcctgccttcactggcagctaccgctgtgaggtgtccaccaaggacaaatttgactgctccaacttcaatctcactgtccacgaggccatgggcaccggagacctggacctcctatcagccttccgccgcacgagcctggctggaggtggtcggcggatcagtgatagccatgaggacactgggattctggacttcagctcactgctgaaaaagagagacagtttccggaccccgagggactcgaagctggaggcaccagcagaggaggacgtgtgggagatcctacggcaggcacccccatctgagtacgagcgcatcgccttccagtacggcgtcactgacctgcgcggcatgctaaagaggctcaagggcatgaggcgcgatgagaagaagagcacagcctttcagaagaagctggagccggcctaccaggtgagcaaaggccacaagatccggctgaccgtggaactggctgaccatgacgctgaggtcaaatggctcaagaatggccaggagatccagatgagcggcagcaagtacatctttgagtccatcggtgccaagcgtaccctgaccatcagccagtgctcattggcggacgacgcagcctaccagtgcgtggtgggtggcgagaagtgtagcacggagctctttgtgaaagagccccctgtgctcatcacgcgccccttggaggaccagctggtgatggtggggcagcgggtggagtttgagtgtgaagtatcggaggagggggcgcaagtcaaatggctgaaggacggggtggagctgacccgggaggagaccttcaaataccggttcaagaaggacgggcagagacaccacctgatcatcaacgaggccatgctggaggacgcggggcactatgcactgtgcactagcgggggccaggcgctggctgagctcattgtgcaggaaaagaagctggaggtgtaccagagcatcgcagacctgatggtgggcgcaaaggaccaggcggtgttcaaatgtgaggtctcagatgagaatgttcggggtgtgtggctgaagaatgggaaggagctggtgcccgacagccgcataaaggtgtcccacatcgggcgggtccacaaactgaccattgacgacgtcacacctgccgacgaggctgactacagctttgtgcccgagggcttcgcctgcaacctgtcagccaagctccacttcatggaggtcaagattgacttcgtacccaggcaggaacctcccaagatccacctggactgcccaggccgcataccagacaccattgtggttgtagctggaaataagctacgtctggacgtccctatctctggggaccctgctcccactgtgatctggcagaaggctatcacgcaggggaataaggccccagccaggccagccccagatgccccagaggacacaggtgacagcgatgagtgggtgtttgacaagaagctgctgtgtgagaccgagggccgggtccgcgtggagaccaccaaggaccgcagcatcttcacggtcgagggggcagagaaggaagatgagggcgtctacacggtcacagtgaagaaccctgtgggcgaggaccaggtcaacctcacagtcaaggtcatcgacgtgccagacgcacctgcggcccccaagatcagcaacgtgggagaggactcctgcacagtacagtgggagccgcctgcctacgatggcgggcagcccatcctgggctacatcctggagcgcaagaagaagaagagctaccggtggatgcggctgaacttcgacctgattcaggagctgagtcatgaagcgcggcgcatgatcgagggcgtggtgtacgagatgcgcgtctacgcggtcaacgccatcggcatgtccaggcccagccctgcctcccagcccttcatgcctatcggtccccccagcgaacccacccacctggcagtagaggacgtctctgacaccacggtctccctcaagtggcggcccccagagcgcgtgggagcaggaggcctggatggctacagcgtggagtactgcccagagggctgctcagagtgggtggctgccctgcaggggctgacagagcacacatcgatactggtgaaggacctgcccacgggggcccggctgcttttccgagtgcgggcacacaatatggcagggcctggagcccctgttaccaccacggagccggtgacagtgcaggagatcctgcaacggccacggcttcagctgcccaggcacctgcgccagaccattcagaagaaggtcggggagcctgtgaaccttctcatccctttccagggcaagccccggcctcaggtgacctggaccaaagaggggcagcccctggcaggcgaggaggtgagcatccgcaacagccccacagacaccatcctgttcatccgggccgctcgccgcgtgcattcaggcacttaccaggtgacggtgcgcattgagaacatggaggacaaggccacgctggtgctgcaggttgttgacaagccaagtcctccccaggatctccgggtgactgacgcctggggtcttaatgtggctctggagtggaagccaccccaggatgtcggcaacacggagctctgggggtacacagtgcagaaagccgacaagaagaccatggagtggttcaccgtcttggagcattaccgccgcacccactgcgtggtgccagagctcatcattggcaatggctactacttccgcgtcttcagccagaatatggttggctttagtgacagagcggccaccaccaaggagcccgtctttatccccagaccaggcatcacctatgagccacccaactataaggccctggacttctccgaggccccaagcttcacccagcccctggtgaaccgctcggtcatcgcgggctacactgctatgctctgctgtgctgtccggggtagccccaagcccaagatttcctggttcaagaatggcctggacctgggagaagacgcccgcttccgcatgttcagcaagcagggagtgttgactctggagattagaaagccctgcccctttgacgggggcatctatgtctgcagggccaccaacttacagggcgaggcacggtgtgagtgccgcctggaggtgcgagtgcctcagtga

SEQ ID NO: 340 - DNA, 1110 bp, Artificial Sequence
  dRNA/arRNA
atgttgaagccatcattaccattcacatccctcttattcctgcagctgcccctgctgggagtggggctgaacacgacaattctgacgcccaatgggaatgaagacaccacagctgatttcttcctgaccactatgcccactgactccctcagtgtttccactctgcccctcccagaggttcagtgttttgtgttcaatgtcgagtacatgaattgcacttggaacagcagctctgagccccagcctaccaacctcactctgcattattggtacaagaactcggataatgataaagtccagaagtgcagccactatctattctctgaagaaatcacttctggctgtcagttgcaaaaaaaggagatccacctctaccaaacatttgttgttcagctccaggacccacgggaacccaggagacaggccacacagatgctaaaactgcagaatctggtgatcccctgggctccagagaacctaacacttcacaaactgagtgaatcccagctagaactgaactggaacaacagattcttgaaccactgtttggagcacttggtgcagtaccggactgactgggaccacagctggactgaacaatcagtggattatagacataagttctccttgcctagtgtggatgggcagaaacgctacacgtttcgtgttcggagccgctttaacccactctgtggaagtgctcagcattggagtgaatggagccacccaatccactgggggagcaatacttcaaaagagaatcctttcctgtttgcattggaagccgtggttatctctgttggctccatgggattgattatcagccttctctgtgtgtatttctggctggaacggacgatgccccgaattcccaccctgaagaacctagaggatcttgttactgaataccacgggaacttttcggcctggagtggtgtgtctaagggactggctgagagtctgcagccagactacagtgaacgactctgcctcgtcagtgagattcccccaaaaggaggggcccttggggaggggcctggggcctccccatgcaaccagcatagcccctactgggcccccccatgttacaccctaaagcctgaaacctga

SEQ ID NO: 341 - RNA, 108 nt, Artificial Sequence
  dRNA/arRNA
uaccgcuacagccacgcugauuucagcuauaccugcccgguauaaagggacguucacaccggauguucuccgcggggauaucgcgauauucaggauuaaaagaagugc

SEQ ID NO: 342 - DNA, 91 bp, Artificial Sequence
  dRNA/arRNA
uaauccugaauaucgcgcaauuccccagcagagaacaucgcggugugaacgucccuuuauaccgggcagguauagcugaaaucagcguggc

SEQ ID NO: 343 - RNA, 71 nt, Artificial Sequence
  dRNA/arRNA
uuucagcuauaccugcccgguauaaagggacguucacaccgcgauguucucugcuggggaauugcgcgaua

SEQ ID NO: 344 - RNA, 91 nt, Artificial Sequence
  dRNA/arRNA
gugugguugcuguccaggacggucccggccugcgacacuucggcccagagcugcuccucaucugcggggcgggggggggccgucgccgcgu

SEQ ID NO: 345 - RNA, 71 nt, Artificial Sequence
  dRNA/arRNA
uguccaggacggucccggccugcgacacuucggcccagagcugcuccucaucugcggggcgggggggggcc

SEQ ID NO: 346 - RNA, 51 nt, Artificial Sequence
  dRNA/arRNA
ggucccggccugcgacacuucggcccagagcugcuccucaucugcggggcg

SEQ ID NO: 347 - RNA, 101 nt, Artificial Sequence
  dRNA/arRNA
gacgcccaccgugugguugcuguccaggacggucccggccugcgacacuucggcccagagcugcuccucaucugcggggcgggggggggccgucgccgcgu

SEQ ID NO: 348 - RNA, 91 nt, Artificial Sequence
  dRNA/arRNA
gacgcccaccgugugguugcuguccaggacggucccggccugcgacacuucggcccagagcugcuccucaucugcggggcgggggggggcc

SEQ ID NO: 349 - RNA, 81 nt, Artificial Sequence
  dRNA/arRNA
gacgcccaccgugugguugcuguccaggacggucccggccugcgacacuucggcccagagcugcuccucaucugcggggcg

SEQ ID NO: 350 - RNA, 71 nt, Artificial Sequence
  dRNA/arRNA
gacgcccaccgugugguugcuguccaggacggucccggccugcgacacuucggcccagagcugcuccucau

SEQ ID NO: 351 - RNA, 61 nt, Artificial Sequence
  dRNA/arRNA
gacgcccaccgugugguugcuguccaggacggucccggccugcgacacuucggcccagagc

SEQ ID NO: 352 - RNA, 101 nt, Artificial Sequence
  dRNA/arRNA
gugugguugcuguccaggacggucccggccugcgacacuucggcccagagcugcuccucaucugcggggcgggggggggccgucgccgcguggggucguug

SEQ ID NO: 353 - RNA, 91 nt, Artificial Sequence
  dRNA/arRNA
uguccaggacggucccggccugcgacacuucggcccagagcugcuccucaucugcggggcgggggggggccgucgccgcguggggucguug

SEQ ID NO: 354 - RNA, 81 nt, Artificial Sequence
  dRNA/arRNA
ggucccggccugcgacacuucggcccagagcugcuccucaucugcggggcgggggggggccgucgccgcguggggucguug

SEQ ID NO: 355 - RNA, 71 nt, Artificial Sequence
  dRNA/arRNA
ugcgacacuucggcccagagcugcuccucaucugcggggcgggggggggccgucgccgcguggggucguug

SEQ ID NO: 356 - RNA, 61 nt, Artificial Sequence
  dRNA/arRNA
cggcccagagcugcuccucaucugcggggcgggggggggccgucgccgcguggggucguug

SEQ ID NO: 357 - RNA, 80 nt, Artificial Sequence
  dRNA/arRNA
gacgcccaccgugugguugcuguccaggacggucccggccugcgacacuucggcccagagcugcuccucaucugcggggc

SEQ ID NO: 358 - RNA, 79 nt, Artificial Sequence
  dRNA/arRNA
gacgcccaccgugugguugcuguccaggacggucccggccugcgacacuucggcccagagcugcuccucaucugcgggg

SEQ ID NO: 359 - RNA, 78 nt, Artificial Sequence
  dRNA/arRNA
gacgcccaccgugugguugcuguccaggacggucccggccugcgacacuucggcccagagcugcuccucaucugcggg

SEQ ID NO: 360 - RNA, 77 nt, Artificial Sequence
  dRNA/arRNA
gacgcccaccgugugguugcuguccaggacggucccggccugcgacacuucggcccagagcugcuccucaucugcgg

SEQ ID NO: 361 - RNA, 76 nt, Artificial Sequence
  dRNA/arRNA
gacgcccaccgugugguugcuguccaggacggucccggccugcgacacuucggcccagagcugcuccucaucugcg

SEQ ID NO: 362 - RNA, 75 nt, Artificial Sequence
  dRNA/arRNA
gacgcccaccgugugguugcuguccaggacggucccggccugcgacacuucggcccagagcugcuccucaucugc

SEQ ID NO: 363 - RNA, 74 nt, Artificial Sequence
  dRNA/arRNA
gacgcccaccgugugguugcuguccaggacggucccggccugcgacacuucggcccagagcugcuccucaucug

SEQ ID NO: 364 - RNA, 73 nt, Artificial Sequence
  dRNA/arRNA
gacgcccaccgugugguugcuguccaggacggucccggccugcgacacuucggcccagagcugcuccucaucu

SEQ ID NO: 365 - RNA, 72 nt, Artificial Sequence
  dRNA/arRNA
gacgcccaccgugugguugcuguccaggacggucccggccugcgacacuucggcccagagcugcuccucauc

SEQ ID NO: 366 - RNA, 70 nt, Artificial Sequence
  dRNA/arRNA
gacgcccaccgugugguugcuguccaggacggucccggccugcgacacuucggcccagagcugcuccuca

SEQ ID NO: 367 - RNA, 69 nt, Artificial Sequence
  dRNA/arRNA
gacgcccaccgugugguugcuguccaggacggucccggccugcgacacuucggcccagagcugcuccuc

SEQ ID NO: 368 - RNA, 68 nt, Artificial Sequence
  dRNA/arRNA
gacgcccaccgugugguugcuguccaggacggucccggccugcgacacuucggcccagagcugcuccu

SEQ ID NO: 369 - RNA, 67 nt, Artificial Sequence
  dRNA/arRNA
gacgcccaccgugugguugcuguccaggacggucccggccugcgacacuucggcccagagcugcucc

SEQ ID NO: 370 - RNA, 66 nt, Artificial Sequence
  dRNA/arRNA
gacgcccaccgugugguugcuguccaggacggucccggccugcgacacuucggcccagagcugcuc

SEQ ID NO: 371 - RNA, 65 nt, Artificial Sequence
  dRNA/arRNA
gacgcccaccgugugguugcuguccaggacggucccggccugcgacacuucggcccagagcugcu

SEQ ID NO: 372 - RNA, 64 nt, Artificial Sequence
  dRNA/arRNA
gacgcccaccgugugguugcuguccaggacggucccggccugcgacacuucggcccagagcugc

SEQ ID NO: 373 - RNA, 63 nt, Artificial Sequence
  dRNA/arRNA
gacgcccaccgugugguugcuguccaggacggucccggccugcgacacuucggcccagagcug

SEQ ID NO: 374 - RNA, 62 nt, Artificial Sequence
  dRNA/arRNA
gacgcccaccgugugguugcuguccaggacggucccggccugcgacacuucggcccagagcu

SEQ ID NO: 375 - RNA, 61 nt, Artificial Sequence; identical to SEQ ID NO: 351
  dRNA/arRNA

SEQ ID NO: 376 - RNA, 70 nt, Artificial Sequence
  dRNA/arRNA
uaccgcuacagccacgcugauuucagcuauaccugcccgguauaaagggacguucacaccgcgauguucu

SEQ ID NO: 377 - RNA, 66 nt, Artificial Sequence
  dRNA/arRNA
uaccgcuacagccacgcugauuucagcuauaccugcccgguauaaagggacguucacaccgcgaug

SEQ ID NO: 378 - RNA, 71 nt, Artificial Sequence
  dRNA/arRNA
ccaccgugugguugcuguccaggacggucccggccugcgacacuucggcccagagcugcuccucaucugcg

SEQ ID NO: 379 - RNA, 66 nt, Artificial Sequence
  dRNA/arRNA
gugugguugcuguccaggacggucccggccugcgacacuucggcccagagcugcuccucaucugcg

SEQ ID NO: 380 - RNA, 61 nt, Artificial Sequence
  dRNA/arRNA
guugcuguccaggacggucccggccugcgacacuucggcccagagcugcuccucaucugcg

SEQ ID NO: 381 - RNA, 56 nt, Artificial Sequence
  dRNA/arRNA
uguccaggacggucccggccugcgacacuucggcccagagcugcuccucaucugcg

SEQ ID NO: 382 - RNA, 66 nt, Artificial Sequence
  dRNA/arRNA
ccaccgugugguugcuguccaggacggucccggccugcgacacuucggcccagagcugcuccucau

SEQ ID NO: 383 - RNA, 61 nt, Artificial Sequence
  dRNA/arRNA
gugugguugcuguccaggacggucccggccugcgacacuucggcccagagcugcuccucau

SEQ ID NO: 384 - RNA, 56 nt, Artificial Sequence
  dRNA/arRNA
guugcuguccaggacggucccggccugcgacacuucggcccagagcugcuccucau

SEQ ID NO: 385 - RNA, 51 nt, Artificial Sequence
  dRNA/arRNA
uguccaggacggucccggccugcgacacuucggcccagagcugcuccucau

SEQ ID NO: 386 - RNA, 67 nt, Artificial Sequence
  dRNA/arRNA
acgcccaccgugugguugcuguccaggacggucccggccugcgacacuucggcccagagcugcuccu

SEQ ID NO: 387 - RNA, 67 nt, Artificial Sequence
  dRNA/arRNA
cgcccaccgugugguugcuguccaggacggucccggccugcgacacuucggcccagagcugcuccuc

SEQ ID NO: 388 - RNA, 67 nt, Artificial Sequence
  dRNA/arRNA
gcccaccgugugguugcuguccaggacggucccggccugcgacacuucggcccagagcugcuccuca

SEQ ID NO: 389 - RNA, 67 nt, Artificial Sequence
  dRNA/arRNA
cccaccgugugguugcuguccaggacggucccggccugcgacacuucggcccagagcugcuccucau

SEQ ID NO: 390 - RNA, 67 nt, Artificial Sequence
  dRNA/arRNA
ccaccgugugguugcuguccaggacggucccggccugcgacacuucggcccagagcugcuccucauc

SEQ ID NO: 391 - RNA, 67 nt, Artificial Sequence
  dRNA/arRNA
caccgugugguugcuguccaggacggucccggccugcgacacuucggcccagagcugcuccucaucu

SEQ ID NO: 392 - RNA, 67 nt, Artificial Sequence
  dRNA/arRNA
accgugugguugcuguccaggacggucccggccugcgacacuucggcccagagcugcuccucaucug

SEQ ID NO: 393 - RNA, 67 nt, Artificial Sequence
  dRNA/arRNA
ccgugugguugcuguccaggacggucccggccugcgacacuucggcccagagcugcuccucaucugc

SEQ ID NO: 394 - RNA, 67 nt, Artificial Sequence
  dRNA/arRNA
cgugugguugcuguccaggacggucccggccugcgacacuucggcccagagcugcuccucaucugcg

SEQ ID NO: 395 - RNA, 67 nt, Artificial Sequence
  dRNA/arRNA
gugugguugcuguccaggacggucccggccugcgacacuucggcccagagcugcuccucaucugcgg

SEQ ID NO: 396 - RNA, 67 nt, Artificial Sequence
  dRNA/arRNA
ugugguugcuguccaggacggucccggccugcgacacuucggcccagagcugcuccucaucugcggg

SEQ ID NO: 397 - RNA, 67 nt, Artificial Sequence
  dRNA/arRNA
gugguugcuguccaggacggucccggccugcgacacuucggcccagagcugcuccucaucugcgggg

SEQ ID NO: 398 - RNA, 70 nt, Artificial Sequence
  dRNA/arRNA
acgcccaccgugugguugcuguccaggacggucccggccugcgacacuucggcccagagcugcuccucau

SEQ ID NO: 399 - RNA, 70 nt, Artificial Sequence
  dRNA/arRNA
cgcccaccgugugguugcuguccaggacggucccggccugcgacacuucggcccagagcugcuccucauc

SEQ ID NO: 400 - RNA, 70 nt, Artificial Sequence
  dRNA/arRNA
gcccaccgugugguugcuguccaggacggucccggccugcgacacuucggcccagagcugcuccucaucu

SEQ ID NO: 401 - RNA, 70 nt, Artificial Sequence
  dRNA/arRNA
cccaccgugugguugcuguccaggacggucccggccugcgacacuucggcccagagcugcuccucaucug

SEQ ID NO: 402 - RNA, 70 nt, Artificial Sequence
  dRNA/arRNA
ccaccgugugguugcuguccaggacggucccggccugcgacacuucggcccagagcugcuccucaucugc

SEQ ID NO: 403 - RNA, 70 nt, Artificial Sequence
  dRNA/arRNA
caccgugugguugcuguccaggacggucccggccugcgacacuucggcccagagcugcuccucaucugcg

SEQ ID NO: 404 - RNA, 70 nt, Artificial Sequence
  dRNA/arRNA
accgugugguugcuguccaggacggucccggccugcgacacuucggcccagagcugcuccucaucugcgg

SEQ ID NO: 405 - RNA, 70 nt, Artificial Sequence
  dRNA/arRNA
ccgugugguugcuguccaggacggucccggccugcgacacuucggcccagagcugcuccucaucugcggg

SEQ ID NO: 406 - RNA, 70 nt, Artificial Sequence
  dRNA/arRNA
cgugugguugcuguccaggacggucccggccugcgacacuucggcccagagcugcuccucaucugcgggg

SEQ ID NO: 407 - RNA, 72 nt, Artificial Sequence
  dRNA/arRNA
acgcccaccgugugguugcuguccaggacggucccggccugcgacacuucggcccagagcugcuccucaucu

SEQ ID NO: 408 - RNA, 72 nt, Artificial Sequence
  dRNA/arRNA
cgcccaccgugugguugcuguccaggacggucccggccugcgacacuucggcccagagcugcuccucaucug

SEQ ID NO: 409 - RNA, 72 nt, Artificial Sequence
  dRNA/arRNA
gcccaccgugugguugcuguccaggacggucccggccugcgacacuucggcccagagcugcuccucaucugc

SEQ ID NO: 410 - RNA, 72 nt, Artificial Sequence
  dRNA/arRNA
cccaccgugugguugcuguccaggacggucccggccugcgacacuucggcccagagcugcuccucaucugcg

SEQ ID NO: 411 - RNA, 72 nt, Artificial Sequence
  dRNA/arRNA
ccaccgugugguugcuguccaggacggucccggccugcgacacuucggcccagagcugcuccucaucugcgg

SEQ ID NO: 412 - RNA, 72 nt, Artificial Sequence
  dRNA/arRNA
caccgugugguugcuguccaggacggucccggccugcgacacuucggcccagagcugcuccucaucugcggg

SEQ ID NO: 413 - RNA, 72 nt, Artificial Sequence
  dRNA/arRNA
accgugugguugcuguccaggacggucccggccugcgacacuucggcccagagcugcuccucaucugcgggg

SEQ ID NO: 414 - RNA, 50 nt, Artificial Sequence
  dRNA/arRNA
cuguccaggacggucccggccugcgacacuucggcccagagcugcuccuc

SEQ ID NO: 415 - DNA, 20 bp, Artificial Sequence
  Forward primer: hIDUA-62F
ccttcctgagctaccacccg

SEQ ID NO: 416 - DNA, 20 bp, Artificial Sequence
  Reverse primer: hIDUA-62R
ccagggctcgaactcggtag